European Patent Specification EP 3 550 958 B1, published June 17, 2026. Title: Methods for Improving Transformation Frequency. Applicant: Syngenta Participations, AG Elumalai, Sivamani Que, Qiudeng Schweiner, Michael. The sequence listing filed with the application follows.

SEQUENCE LISTING (35 sequences)

SEQ ID NO: 1 - DNA, 552 bp, Artificial Sequence
  derived from Streptomyces viridochromogenes
atgtccccggagcgccgcccggtggagatccgcccggccaccgccgccgacatggccgccgtgtgcgacatcgtgaaccactacatcgagacctccaccgtgaacttccgcaccgagccgcagaccccgcaggagtggatcgacgacctcgagcgcctccaggaccgctacccgtggctcgtggccgaggtggagggcgtggtggccggcatcgcctacgccggcccgtggaaggcccgcaacgcctacgactggaccgtggagtccaccgtgtacgtgtcccaccgccaccagcgcctcggcctcggctccaccctctacacccacctcctcaagtctatggaggcccagggcttcaagtccgtggtggccgtgatcggcctcccgaacgacccgtccgtgcgcctccacgaggccctcggctacaccgcccgcggcaccctgcgcgccgccggctacaagcacggcggctggcacgacgtgggcttctggcagcgcgacttcgagctgccggccccgccgcgcccggtgcgcccggtgacccagatttga

SEQ ID NO: 2 - DNA, 5552 bp, Artificial Sequence
  derived from Streptomyces viridochromogenes and Zea mays
ggaaaaccaaaacaacgaataagcaaactgcaggaaaagtatgcagtggaaaccaacccagattcggacgataggaaagtatcaagtgaatgatttgccaggaaaaggagaggggtaaaaaggggcgaagatttagaagatctaaagcacaagaaccagagattagattgaacaatagggaacttggagcatcctttttttcttcagggaaaaactgaaaatccaaaccatgttgagcaaaaccgagtgggattggaaaccaaaaaacccgagataaagaaactcgagaaaaagcatgaaatcgaaaccaacttcagtaaaacaaaaggaggacagaaaagaaagtcggaagctataaagaatacattaacattcagtgaaacagcatgctgtcttcttctttttttatgcacaacagagcatacatatataccttcccaggctgaggacttggcggaggagagccgcggataggttggcggtgcagacggtctggacgggcccgaagacggagacgaacagcgggcccttcctgcccaggcaccacgcttggaacgccaagcacgcgccaaccgcggccccgccgaggacgacgatccccgcgacaagcgtggcgtcgatcctgggcgaccccaagccgaggaacctcccttccaggacgagccgtaggacggcggtgagagaggcacccgtcgcggaggtggcgcagcacaaggtgagcagcgcggggaaggcggcgagcgtggcggcctgcaggacggtgacgagcgcgaagacggtgacgccggcgacgaggcagcagcagccgaggttccagtcgtaggaggaagccggaccaaaccgggcaatgcaacctgcagatgcactagacggaggtaacgaggaggaggagaaaacagagcaagagcaggcggagagaagatagagcaaaacacgagtgaggcacagcgtaagcactcggtagaagtctccagaggcgaggtgcgcacaggagaacagatgagtaaagtcagccaaggatgcacgatccaacggctacgaatttttggagtgacgtggataggctcaaaggcgccatttccatccggctttatagtattttaaaaaaattcattttcctccctctagtgtgtgcggaggcgtgagcccgtttaacggcgttgagaagtctaacggacaccaaccacaaccaggaaccagcgccggccgcgccgccgagtgaagcagactgcatacggcacggcgcggcatctctctggctgcctctcgagagttccgcccccaccttcccgcggtagcgtggtggtttcgctttccgctgtcggcatccggaagttgcgtggcagagtggacggagacgaggccgggtcctccagctcctctcaaacgtcacggcaccggcatccggcagccagcgcggtccttcccaaccactcgttcccaacccatcccccttcctcgcccgccgtcataaatagccagccccatccccagcttctttccccaacctcatcttctctccttttgctctgaacgcacacaccgcccggtctccgatctccgatccccgatcccctcgtcgatcctaggtacggcgaccatcctaccccccccccccccccctctctctctgccttctctagatcggcgatccgatccatgcttacttggttagggcctgctaactatgttcatgtttgcgttagatccgtgcatggacgcgatctgtacacaccagacgcgttctgattgctagctaactcgccagtacctgggaatcctgggatggctgtagccggccccgcacgcagacgggaccgatttcatgattctctatttttttctttgtttcgttgcctagggtttcgttcgatcgatccgcgttattctttatttccatatattctggtacgatgttgatacggttcgaccgtgctgcttacgttctgtgcgcttgtttgccgggtcatttttaccttgccttttttgtatggtttggttgtggcgatgtggtctggtcgggctgtcgttctagatcggagtagagtgctgtttcaaactgtctagcggatctattagatttggatctgcatgtgtgacatatatcttcgtagttaagatgatgcatctgtatgtgtgacatgcggatctattagatttggatctgtatgtgtgacatatatcttcgtagttgagatgatgcatctgtatgtgtgacatatatcttcgtagttaagattatgcatggaaatatcaatcctttagataaggacgggtatacttgttgctgtgggttttactggtacttcgatagatgcatatacatgatctaacatgcttagatacatgaagtaacatgctgctacggtttaataattcttgagttgatttttactggtacttagatagatgtatatacatgcttagatacatgaagtaacatgctcctacagttcctttaatcattattgagtacctatatattctaataaatcagtatgttttaaattattttgattttactggtacttagatagatgtatatatacatgctcaaacatgcttagatacatgaagtaacatgctgctacggtttagtcattattgagtgcctatatattctaataaatcagtatgttttaaattattttgattttactggtacttagatagatgtatatatacatgctcaaacatgcttagatacatgaagtaatatgctactacggtttaattgttcttgagtacctatatattctaataaatcagtatgttttaaattatttcgattttactggtacttagatagatgtatatatacatgcttagatacatgaagtaacatgctactacggtttaattgttcttgaatacctatatattctaataaatcagtatgttttaaattatttcgattttactggtacttagatagatgtatatatacatgctcgaacatgcttagatacatgaagtaacatgctacatatatattataataaatcagtatgtcttaaattattttgattttactggtacttagatagatgtatatacatgctcaaacatgcttagatacatgaagtaacatgctactacggtttaatcattattgagtacctatatattctaataaatcagtatgttttcaattgttttgattttactggtacttagatatatgtatatatacatgctcgaacatgcttagatacgtgaagtaacatgctactatggttaattgttcttgagtacctatatattctaataaatcagtatgttttaaattatttcgattttactggtacttagatagatgtatatatacatgctcgaacatgcttagatacatgaagtaacatgctactacggtttaatcgttcttgagtacctatatattctaataaatcagtatgtcttaaattatcttgattttactggtacttagatagatgtatatacatgcttagatacatgaagtaacatgctactatgatttaatcgttcttgagtacctatatattctaataaatcagtatgtttttaattattttgattttactggtacttagatagatgtatatatacatgctcgaacatgcttagatacatgaagtaacatgctactacggtttaatcattcttgagtacctatatattctaataaatcagtatgtttttaattattttgatattactggtacttaacatgtttagatacatcatatagcatgcacatgctgctactgtttaatcattcgtgaatacctatatattctaatatatcagtatgtcttctaattattatgattttgatgtacttgtatggtggcatatgctgcagctatgtgtagattttgaatacccagtgtgatgagcatgcatggcgccttcatagttcatatgctgtttatttcctttgagactgttcttttttgttgatagtcaccctgttgtttggtgattcttatccagatccagatcttcgagatcctaaaccatgtccccggagcgccgcccggtggagatccgcccggccaccgccgccgacatggccgccgtgtgcgacatcgtgaaccactacatcgagacctccaccgtgaacttccgcaccgagccgcagaccccgcaggagtggatcgacgacctcgagcgcctccaggaccgctacccgtggctcgtggccgaggtggagggcgtggtggccggcatcgcctacgccggcccgtggaaggcccgcaacgcctacgactggaccgtggagtccaccgtgtacgtgtcccaccgccaccagcgcctcggcctcggctccaccctctacacccacctcctcaagtctatggaggcccagggcttcaagtccgtggtggccgtgatcggcctcccgaacgacccgtccgtgcgcctccacgaggccctcggctacaccgcccgcggcaccctgcgcgccgccggctacaagcacggcggctggcacgacgtgggcttctggcagcgcgacttcgagctgccggccccgccgcgcccggtgcgcccggtgacccagatttgagccaaggttcaattaagctgctgctgtacctgggtatctgcgtcgtctggtgccctctggtgtacctctatatggatctcgtcgtctaataaacatctgtggtttgtgtgtcatcaatcgtggttgtggcttcgttggtttaatggacctgttgtgtcctctgtgttgtacccaaaactcttctgcagcagtatggcttgaatccttatgaagtttgatatttgaacttaaaagtctgctcattatgtttttttctggttatatctcctaattaactgcctgggatcaaatttgattcgctggtgtttattggacccctcccaggttcttgctttctaccgtttcttgctgaatgttaacttgattctgtcaggctcagtttcccactatggcttacagcttaacgtgtttggtttgttgaatgttaacttggttttgtcaagctcagttttttactctggcttacagcataacatgtttgacttttggttttgctgctttgttattgggttctgggtagttcttgatgaatccaaaagatcatgtgcacagccatattatctatttaagcgatccaggttattactatgaaaggatgccttctagctaaggagtagttaggttttttcttcaaggttaaattttctcgatgctctagtgttcctgtgaccataatcataataattcctttgaaagctctatggtccctggaagcagggcatacaatgcaagacagcaacttgatcacatcaactgaagtatacagggttctcttaactcttggtgacttcggtttaatggaccggttgtactcgtgttctatccgtaaccgttgtgatgtcttgtgtgtttggttgcgggatagctgggaccacgacgtttccgtctaattctgatggatagctatagacggcactgagatggttatattataacctctgatcctgaactctacgagatcgtctcatccgtcattgccaccaaatacaccattaaatta

SEQ ID NO: 3 - DNA, 5527 bp, Artificial Sequence
  derived from Streptomyces viridochromogenes and Zea mays
ggaaaaccaaaacaacgaataagcaaactgcaggaaaagtatgcagtggaaaccaacccagattcggacgataggaaagtatcaagtgaatgatttgccaggaaaaggagaggggtaaaaaggggcgaagatttagaagatctaaagcacaagaaccagagattagattgaacaatagggaacttggagcatcctttttttcttcagggaaaaactgaaaatccaaaccatgttgagcaaaaccgagtgggattggaaaccaaaaaacccgagataaagaaactcgagaaaaagcatgaaatcgaaaccaacttcagtaaaacaaaaggaggacagaaaagaaagtcggaagctataaagaatacattaacattcagtgaaacagcatgctgtcttcttctttttttatgcacaacagagcatacatatataccttcccaggctgaggacttggcggaggagagccgcggataggttggcggtgcagacggtctggacgggcccgaagacggagacgaacagcgggcccttcctgcccaggcaccacgcttggaacgccaagcacgcgccaaccgcggccccgccgaggacgacgatccccgcgacaagcgtggcgtcgatcctgggcgaccccaagccgaggaacctcccttccaggacgagccgtaggacggcggtgagagaggcacccgtcgcggaggtggcgcagcacaaggtgagcagcgcggggaaggcggcgagcgtggcggcctgcaggacggtgacgagcgcgaagacggtgacgccggcgacgaggcagcagcagccgaggttccagtcgtaggaggaagccggaccaaaccgggcaatgcaacctgcagatgcactagacggaggtaacgaggaggaggagaaaacagagcaagagcaggcggagagaagatagagcaaaacacgagtgaggcacagcgtaagcactcggtagaagtctccagaggcgaggtgcgcacaggagaacagatgagtaaagtcagccaaggatgcacgatccaacggctacgaatttttggagtgacgtggataggctcaaaggcgccatttccatccggctttatagtattttaaaaaaattcattttcctccctctagtgtgtgcggaggcgtgagcccgtttaacggcgttgagaagtctaacggacaccaaccacaaccaggaaccagcgccggccgcgccgccgagtgaagcagactgcatacggcacggcgcggcatctctctggctgcctctcgagagttccgcccccaccttcccgcggtagcgtggtggtttcgctttccgctgtcggcatccggaagttgcgtggcagagtggacggagacgaggccgggtcctccagctcctctcaaacgtcacggcaccggcatccggcagccagcgcggtccttcccaaccactcgttcccaacccatcccccttcctcgcccgccgtcataaatagccagccccatccccagcttctttccccaacctcatcttctctccttttgctctgaacgcacacaccgcccggtctccgatctccgatccccgatcccctcgtcgatcctaggtacggcgaccatcctaccccccccccccccccctctctctctgccttctctagatcggcgatccgatccatgcttacttggttagggcctgctaactatgttcatgtttgcgttagatccgtgcatggacgcgatctgtacacaccagacgcgttctgattgctagctaactcgccagtacctgggaatcctgggatggctgtagccggccccgcacgcagacgggaccgatttcatgattctctatttttttctttgtttcgttgcctagggtttcgttcgatcgatccgcgttattctttatttccatatattctggtacgatgttgatacggttcgaccgtgctgcttacgttctgtgcgcttgtttgccgggtcatttttaccttgccttttttgtatggtttggttgtggcgatgtggtctggtcgggctgtcgttctagatcggagtagagtgctgtttcaaactgtctagcggatctattagatttggatctgcatgtgtgacatatatcttcgtagttaagatgatgcatctgtatgtgtgacatgcggatctattagatttggatctgtatgtgtgacatatatcttcgtagttgagatgatgcatctgtatgtgtgacatatatcttcgtagttaagattatgcatggaaatatcaatcctttagataaggacgggtatacttgttgctgtgggttttactggtacttcgatagatgcatatacatgatctaacatgcttagatacatgaagtaacatgctgctacggtttaataattcttgagttgatttttactggtacttagatagatgtatatacatgcttagatacatgaagtaacatgctcctacagttcctttaatcattattgagtacctatatattctaataaatcagtatgttttaaattattttgattttactggtacttagatagatgtatatatacatgctcaaacatgcttagatacatgaagtaacatgctgctacggtttagtcattattgagtgcctatatattctaataaatcagtatgttttaaattattttgattttactggtacttagatagatgtatatatacatgctcaaacatgcttagatacatgaagtaatatgctactacggtttaattgttcttgagtacctatatattctaataaatcagtatgttttaaattatttcgattttactggtacttagatagatgtatatatacatgcttagatacatgaagtaacatgctactacggtttaattgttcttgaatacctatatattctaataaatcagtatgttttaaattatttcgattttactggtacttagatagatgtatatatacatgctcgaacatgcttagatacatgaagtaacatgctacatatatattataataaatcagtatgtcttaaattattttgattttactggtacttagatagatgtatatacatgctcaaacatgcttagatacatgaagtaacatgctactacggtttaatcattattgagtacctatatattctaataaatcagtatgttttcaattgttttgattttactggtacttagatatatgtatatatacatgctcgaacatgcttagatacgtgaagtaacatgctactatggttaattgttcttgagtacctatatattctaataaatcagtatgttttaaattatttcgattttactggtacttagatagatgtatatatacatgctcgaacatgcttagatacatgaagtaacatgctactacggtttaatcgttcttgagtacctatatattctaataaatcagtatgtcttaaattatcttgattttactggtacttagatagatgtatatacatgcttagatacatgaagtaacatgctactatgatttaatcgttcttgagtacctatatattctaataaatcagtatgtttttaattattttgattttactggtacttagatagatgtatatatacatgctcgaacatgcttagatacatgaagtaacatgctactacggtttaatcattcttgagtacctatatattctaataaatcagtatgtttttaattattttgatattactggtacttaacatgtttagatacatcatatagcatgcacatgctgctactgtttaatcattcgtgaatacctatatattctaatatatcagtatgtcttctaattattatgattttgatgtacttgtatggtggcatatgctgcagctatgtgtagattttgaatacccagtgtgatgagcatgcatggcgccttcatagttcatatgctgtttatttcctttgagactgttcttttttgttgatagtcaccctgttgtttggtgattcttatccagatgtccccggagcgccgcccggtggagatccgcccggccaccgccgccgacatggccgccgtgtgcgacatcgtgaaccactacatcgagacctccaccgtgaacttccgcaccgagccgcagaccccgcaggagtggatcgacgacctcgagcgcctccaggaccgctacccgtggctcgtggccgaggtggagggcgtggtggccggcatcgcctacgccggcccgtggaaggcccgcaacgcctacgactggaccgtggagtccaccgtgtacgtgtcccaccgccaccagcgcctcggcctcggctccaccctctacacccacctcctcaagtctatggaggcccagggcttcaagtccgtggtggccgtgatcggcctcccgaacgacccgtccgtgcgcctccacgaggccctcggctacaccgcccgcggcaccctgcgcgccgccggctacaagcacggcggctggcacgacgtgggcttctggcagcgcgacttcgagctgccggccccgccgcgcccggtgcgcccggtgacccagatttgagccaaggttcaattaagctgctgctgtacctgggtatctgcgtcgtctggtgccctctggtgtacctctatatggatctcgtcgtctaataaacatctgtggtttgtgtgtcatcaatcgtggttgtggcttcgttggtttaatggacctgttgtgtcctctgtgttgtacccaaaactcttctgcagcagtatggcttgaatccttatgaagtttgatatttgaacttaaaagtctgctcattatgtttttttctggttatatctcctaattaactgcctgggatcaaatttgattcgctggtgtttattggacccctcccaggttcttgctttctaccgtttcttgctgaatgttaacttgattctgtcaggctcagtttcccactatggcttacagcttaacgtgtttggtttgttgaatgttaacttggttttgtcaagctcagttttttactctggcttacagcataacatgtttgacttttggttttgctgctttgttattgggttctgggtagttcttgatgaatccaaaagatcatgtgcacagccatattatctatttaagcgatccaggttattactatgaaaggatgccttctagctaaggagtagttaggttttttcttcaaggttaaattttctcgatgctctagtgttcctgtgaccataatcataataattcctttgaaagctctatggtccctggaagcagggcatacaatgcaagacagcaacttgatcacatcaactgaagtatacagggttctcttaactcttggtgacttcggtttaatggaccggttgtactcgtgttctatccgtaaccgttgtgatgtcttgtgtgtttggttgcgggatagctgggaccacgacgtttccgtctaattctgatggatagctatagacggcactgagatggttatattataacctctgatcctgaactctacgagatcgtctcatccgtcattgccaccaaatacaccattaaatta

SEQ ID NO: 4 - DNA, 6067 bp, Artificial Sequence
  derived from Streptomyces viridochromogenes and Zea mays
agctgcttgtggggaccagacaaaaaaggaatggtgcagaattgttaggcgcacctaccaaaagcaactttgcctttattgcaaagataaagcagattcctctagtacaagtggggaacaaaataacgtggaaaagagctgtcctgacagcccactcactattgcgtttgacgaacgcagtgacgaccacaaaactcgagacttttcaacaaagggtattatccggaaacctcctcggattccattgcccagctatctgtcactttattgtgaagatagtggaaaaggaaggtggctcctacaaatgccatcattgcgataaaggaaaggctatcgttgaagatgcctctgccgacagtggtcccaaagatggacccccacccacgaggagcatcgtggaaaaagaagacgttccaaccacgtcttcaaagcaagtggattgatgtgatatctccactgacgtaagggttgacgaacaatcccactatccttctgcctaattagctaacggacccggaaaaccaaaacaacgaataagcaaactgcaggaaaagtatgcagtggaaaccaacccagattcggacgataggaaagtatcaagtgaatgatttgccaggaaaaggagaggggtaaaaaggggcgaagatttagaagatctaaagcacaagaaccagagattagattgaacaatagggaacttggagcatcctttttttcttcagggaaaaactgaaaatccaaaccatgttgagcaaaaccgagtgggattggaaaccaaaaaacccgagataaagaaactcgagaaaaagcatgaaatcgaaaccaacttcagtaaaacaaaaggaggacagaaaagaaagtcggaagctataaagaatacattaacattcagtgaaacagcatgctgtcttcttctttttttatgcacaacagagcatacatatataccttcccaggctgaggacttggcggaggagagccgcggataggttggcggtgcagacggtctggacgggcccgaagacggagacgaacagcgggcccttcctgcccaggcaccacgcttggaacgccaagcacgcgccaaccgcggccccgccgaggacgacgatccccgcgacaagcgtggcgtcgatcctgggcgaccccaagccgaggaacctcccttccaggacgagccgtaggacggcggtgagagaggcacccgtcgcggaggtggcgcagcacaaggtgagcagcgcggggaaggcggcgagcgtggcggcctgcaggacggtgacgagcgcgaagacggtgacgccggcgacgaggcagcagcagccgaggttccagtcgtaggaggaagccggaccaaaccgggcaatgcaacctgcagatgcactagacggaggtaacgaggaggaggagaaaacagagcaagagcaggcggagagaagatagagcaaaacacgagtgaggcacagcgtaagcactcggtagaagtctccagaggcgaggtgcgcacaggagaacagatgagtaaagtcagccaaggatgcacgatccaacggctacgaatttttggagtgacgtggataggctcaaaggcgccatttccatccggctttatagtattttaaaaaaattcattttcctccctctagtgtgtgcggaggcgtgagcccgtttaacggcgttgagaagtctaacggacaccaaccacaaccaggaaccagcgccggccgcgccgccgagtgaagcagactgcatacggcacggcgcggcatctctctggctgcctctcgagagttccgcccccaccttcccgcggtagcgtggtggtttcgctttccgctgtcggcatccggaagttgcgtggcagagtggacggagacgaggccgggtcctccagctcctctcaaacgtcacggcaccggcatccggcagccagcgcggtccttcccaaccactcgttcccaacccatcccccttcctcgcccgccgtcataaatagccagccccatccccagcttctttccccaacctcatcttctctccttttgctctgaacgcacacaccgcccggtctccgatctccgatccccgatcccctcgtcgatcctaggtacggcgaccatcctaccccccccccccccccctctctctctgccttctctagatcggcgatccgatccatgcttacttggttagggcctgctaactatgttcatgtttgcgttagatccgtgcatggacgcgatctgtacacaccagacgcgttctgattgctagctaactcgccagtacctgggaatcctgggatggctgtagccggccccgcacgcagacgggaccgatttcatgattctctatttttttctttgtttcgttgcctagggtttcgttcgatcgatccgcgttattctttatttccatatattctggtacgatgttgatacggttcgaccgtgctgcttacgttctgtgcgcttgtttgccgggtcatttttaccttgccttttttgtatggtttggttgtggcgatgtggtctggtcgggctgtcgttctagatcggagtagagtgctgtttcaaactgtctagcggatctattagatttggatctgcatgtgtgacatatatcttcgtagttaagatgatgcatctgtatgtgtgacatgcggatctattagatttggatctgtatgtgtgacatatatcttcgtagttgagatgatgcatctgtatgtgtgacatatatcttcgtagttaagattatgcatggaaatatcaatcctttagataaggacgggtatacttgttgctgtgggttttactggtacttcgatagatgcatatacatgatctaacatgcttagatacatgaagtaacatgctgctacggtttaataattcttgagttgatttttactggtacttagatagatgtatatacatgcttagatacatgaagtaacatgctcctacagttcctttaatcattattgagtacctatatattctaataaatcagtatgttttaaattattttgattttactggtacttagatagatgtatatatacatgctcaaacatgcttagatacatgaagtaacatgctgctacggtttagtcattattgagtgcctatatattctaataaatcagtatgttttaaattattttgattttactggtacttagatagatgtatatatacatgctcaaacatgcttagatacatgaagtaatatgctactacggtttaattgttcttgagtacctatatattctaataaatcagtatgttttaaattatttcgattttactggtacttagatagatgtatatatacatgcttagatacatgaagtaacatgctactacggtttaattgttcttgaatacctatatattctaataaatcagtatgttttaaattatttcgattttactggtacttagatagatgtatatatacatgctcgaacatgcttagatacatgaagtaacatgctacatatatattataataaatcagtatgtcttaaattattttgattttactggtacttagatagatgtatatacatgctcaaacatgcttagatacatgaagtaacatgctactacggtttaatcattattgagtacctatatattctaataaatcagtatgttttcaattgttttgattttactggtacttagatatatgtatatatacatgctcgaacatgcttagatacgtgaagtaacatgctactatggttaattgttcttgagtacctatatattctaataaatcagtatgttttaaattatttcgattttactggtacttagatagatgtatatatacatgctcgaacatgcttagatacatgaagtaacatgctactacggtttaatcgttcttgagtacctatatattctaataaatcagtatgtcttaaattatcttgattttactggtacttagatagatgtatatacatgcttagatacatgaagtaacatgctactatgatttaatcgttcttgagtacctatatattctaataaatcagtatgtttttaattattttgattttactggtacttagatagatgtatatatacatgctcgaacatgcttagatacatgaagtaacatgctactacggtttaatcattcttgagtacctatatattctaataaatcagtatgtttttaattattttgatattactggtacttaacatgtttagatacatcatatagcatgcacatgctgctactgtttaatcattcgtgaatacctatatattctaatatatcagtatgtcttctaattattatgattttgatgtacttgtatggtggcatatgctgcagctatgtgtagattttgaatacccagtgtgatgagcatgcatggcgccttcatagttcatatgctgtttatttcctttgagactgttcttttttgttgatagtcaccctgttgtttggtgattcttatccagatccagatcttcgagatcctaaaccatgtccccggagcgccgcccggtggagatccgcccggccaccgccgccgacatggccgccgtgtgcgacatcgtgaaccactacatcgagacctccaccgtgaacttccgcaccgagccgcagaccccgcaggagtggatcgacgacctcgagcgcctccaggaccgctacccgtggctcgtggccgaggtggagggcgtggtggccggcatcgcctacgccggcccgtggaaggcccgcaacgcctacgactggaccgtggagtccaccgtgtacgtgtcccaccgccaccagcgcctcggcctcggctccaccctctacacccacctcctcaagtctatggaggcccagggcttcaagtccgtggtggccgtgatcggcctcccgaacgacccgtccgtgcgcctccacgaggccctcggctacaccgcccgcggcaccctgcgcgccgccggctacaagcacggcggctggcacgacgtgggcttctggcagcgcgacttcgagctgccggccccgccgcgcccggtgcgcccggtgacccagatttgagccaaggttcaattaagctgctgctgtacctgggtatctgcgtcgtctggtgccctctggtgtacctctatatggatctcgtcgtctaataaacatctgtggtttgtgtgtcatcaatcgtggttgtggcttcgttggtttaatggacctgttgtgtcctctgtgttgtacccaaaactcttctgcagcagtatggcttgaatccttatgaagtttgatatttgaacttaaaagtctgctcattatgtttttttctggttatatctcctaattaactgcctgggatcaaatttgattcgctggtgtttattggacccctcccaggttcttgctttctaccgtttcttgctgaatgttaacttgattctgtcaggctcagtttcccactatggcttacagcttaacgtgtttggtttgttgaatgttaacttggttttgtcaagctcagttttttactctggcttacagcataacatgtttgacttttggttttgctgctttgttattgggttctgggtagttcttgatgaatccaaaagatcatgtgcacagccatattatctatttaagcgatccaggttattactatgaaaggatgccttctagctaaggagtagttaggttttttcttcaaggttaaattttctcgatgctctagtgttcctgtgaccataatcataataattcctttgaaagctctatggtccctggaagcagggcatacaatgcaagacagcaacttgatcacatcaactgaagtatacagggttctcttaactcttggtgacttcggtttaatggaccggttgtactcgtgttctatccgtaaccgttgtgatgtcttgtgtgtttggttgcgggatagctgggaccacgacgtttccgtctaattctgatggatagctatagacggcactgagatggttatattataacctctgatcctgaactctacgagatcgtctcatccgtcattgccaccaaatacaccattaaatta

SEQ ID NO: 5 - DNA, 6042 bp, Artificial Sequence
  derived from Streptomyces viridochromogenes and Zea mays
agctgcttgtggggaccagacaaaaaaggaatggtgcagaattgttaggcgcacctaccaaaagcaactttgcctttattgcaaagataaagcagattcctctagtacaagtggggaacaaaataacgtggaaaagagctgtcctgacagcccactcactattgcgtttgacgaacgcagtgacgaccacaaaactcgagacttttcaacaaagggtattatccggaaacctcctcggattccattgcccagctatctgtcactttattgtgaagatagtggaaaaggaaggtggctcctacaaatgccatcattgcgataaaggaaaggctatcgttgaagatgcctctgccgacagtggtcccaaagatggacccccacccacgaggagcatcgtggaaaaagaagacgttccaaccacgtcttcaaagcaagtggattgatgtgatatctccactgacgtaagggttgacgaacaatcccactatccttctgcctaattagctaacggacccggaaaaccaaaacaacgaataagcaaactgcaggaaaagtatgcagtggaaaccaacccagattcggacgataggaaagtatcaagtgaatgatttgccaggaaaaggagaggggtaaaaaggggcgaagatttagaagatctaaagcacaagaaccagagattagattgaacaatagggaacttggagcatcctttttttcttcagggaaaaactgaaaatccaaaccatgttgagcaaaaccgagtgggattggaaaccaaaaaacccgagataaagaaactcgagaaaaagcatgaaatcgaaaccaacttcagtaaaacaaaaggaggacagaaaagaaagtcggaagctataaagaatacattaacattcagtgaaacagcatgctgtcttcttctttttttatgcacaacagagcatacatatataccttcccaggctgaggacttggcggaggagagccgcggataggttggcggtgcagacggtctggacgggcccgaagacggagacgaacagcgggcccttcctgcccaggcaccacgcttggaacgccaagcacgcgccaaccgcggccccgccgaggacgacgatccccgcgacaagcgtggcgtcgatcctgggcgaccccaagccgaggaacctcccttccaggacgagccgtaggacggcggtgagagaggcacccgtcgcggaggtggcgcagcacaaggtgagcagcgcggggaaggcggcgagcgtggcggcctgcaggacggtgacgagcgcgaagacggtgacgccggcgacgaggcagcagcagccgaggttccagtcgtaggaggaagccggaccaaaccgggcaatgcaacctgcagatgcactagacggaggtaacgaggaggaggagaaaacagagcaagagcaggcggagagaagatagagcaaaacacgagtgaggcacagcgtaagcactcggtagaagtctccagaggcgaggtgcgcacaggagaacagatgagtaaagtcagccaaggatgcacgatccaacggctacgaatttttggagtgacgtggataggctcaaaggcgccatttccatccggctttatagtattttaaaaaaattcattttcctccctctagtgtgtgcggaggcgtgagcccgtttaacggcgttgagaagtctaacggacaccaaccacaaccaggaaccagcgccggccgcgccgccgagtgaagcagactgcatacggcacggcgcggcatctctctggctgcctctcgagagttccgcccccaccttcccgcggtagcgtggtggtttcgctttccgctgtcggcatccggaagttgcgtggcagagtggacggagacgaggccgggtcctccagctcctctcaaacgtcacggcaccggcatccggcagccagcgcggtccttcccaaccactcgttcccaacccatcccccttcctcgcccgccgtcataaatagccagccccatccccagcttctttccccaacctcatcttctctccttttgctctgaacgcacacaccgcccggtctccgatctccgatccccgatcccctcgtcgatcctaggtacggcgaccatcctaccccccccccccccccctctctctctgccttctctagatcggcgatccgatccatgcttacttggttagggcctgctaactatgttcatgtttgcgttagatccgtgcatggacgcgatctgtacacaccagacgcgttctgattgctagctaactcgccagtacctgggaatcctgggatggctgtagccggccccgcacgcagacgggaccgatttcatgattctctatttttttctttgtttcgttgcctagggtttcgttcgatcgatccgcgttattctttatttccatatattctggtacgatgttgatacggttcgaccgtgctgcttacgttctgtgcgcttgtttgccgggtcatttttaccttgccttttttgtatggtttggttgtggcgatgtggtctggtcgggctgtcgttctagatcggagtagagtgctgtttcaaactgtctagcggatctattagatttggatctgcatgtgtgacatatatcttcgtagttaagatgatgcatctgtatgtgtgacatgcggatctattagatttggatctgtatgtgtgacatatatcttcgtagttgagatgatgcatctgtatgtgtgacatatatcttcgtagttaagattatgcatggaaatatcaatcctttagataaggacgggtatacttgttgctgtgggttttactggtacttcgatagatgcatatacatgatctaacatgcttagatacatgaagtaacatgctgctacggtttaataattcttgagttgatttttactggtacttagatagatgtatatacatgcttagatacatgaagtaacatgctcctacagttcctttaatcattattgagtacctatatattctaataaatcagtatgttttaaattattttgattttactggtacttagatagatgtatatatacatgctcaaacatgcttagatacatgaagtaacatgctgctacggtttagtcattattgagtgcctatatattctaataaatcagtatgttttaaattattttgattttactggtacttagatagatgtatatatacatgctcaaacatgcttagatacatgaagtaatatgctactacggtttaattgttcttgagtacctatatattctaataaatcagtatgttttaaattatttcgattttactggtacttagatagatgtatatatacatgcttagatacatgaagtaacatgctactacggtttaattgttcttgaatacctatatattctaataaatcagtatgttttaaattatttcgattttactggtacttagatagatgtatatatacatgctcgaacatgcttagatacatgaagtaacatgctacatatatattataataaatcagtatgtcttaaattattttgattttactggtacttagatagatgtatatacatgctcaaacatgcttagatacatgaagtaacatgctactacggtttaatcattattgagtacctatatattctaataaatcagtatgttttcaattgttttgattttactggtacttagatatatgtatatatacatgctcgaacatgcttagatacgtgaagtaacatgctactatggttaattgttcttgagtacctatatattctaataaatcagtatgttttaaattatttcgattttactggtacttagatagatgtatatatacatgctcgaacatgcttagatacatgaagtaacatgctactacggtttaatcgttcttgagtacctatatattctaataaatcagtatgtcttaaattatcttgattttactggtacttagatagatgtatatacatgcttagatacatgaagtaacatgctactatgatttaatcgttcttgagtacctatatattctaataaatcagtatgtttttaattattttgattttactggtacttagatagatgtatatatacatgctcgaacatgcttagatacatgaagtaacatgctactacggtttaatcattcttgagtacctatatattctaataaatcagtatgtttttaattattttgatattactggtacttaacatgtttagatacatcatatagcatgcacatgctgctactgtttaatcattcgtgaatacctatatattctaatatatcagtatgtcttctaattattatgattttgatgtacttgtatggtggcatatgctgcagctatgtgtagattttgaatacccagtgtgatgagcatgcatggcgccttcatagttcatatgctgtttatttcctttgagactgttcttttttgttgatagtcaccctgttgtttggtgattcttatccagatgtccccggagcgccgcccggtggagatccgcccggccaccgccgccgacatggccgccgtgtgcgacatcgtgaaccactacatcgagacctccaccgtgaacttccgcaccgagccgcagaccccgcaggagtggatcgacgacctcgagcgcctccaggaccgctacccgtggctcgtggccgaggtggagggcgtggtggccggcatcgcctacgccggcccgtggaaggcccgcaacgcctacgactggaccgtggagtccaccgtgtacgtgtcccaccgccaccagcgcctcggcctcggctccaccctctacacccacctcctcaagtctatggaggcccagggcttcaagtccgtggtggccgtgatcggcctcccgaacgacccgtccgtgcgcctccacgaggccctcggctacaccgcccgcggcaccctgcgcgccgccggctacaagcacggcggctggcacgacgtgggcttctggcagcgcgacttcgagctgccggccccgccgcgcccggtgcgcccggtgacccagatttgagccaaggttcaattaagctgctgctgtacctgggtatctgcgtcgtctggtgccctctggtgtacctctatatggatctcgtcgtctaataaacatctgtggtttgtgtgtcatcaatcgtggttgtggcttcgttggtttaatggacctgttgtgtcctctgtgttgtacccaaaactcttctgcagcagtatggcttgaatccttatgaagtttgatatttgaacttaaaagtctgctcattatgtttttttctggttatatctcctaattaactgcctgggatcaaatttgattcgctggtgtttattggacccctcccaggttcttgctttctaccgtttcttgctgaatgttaacttgattctgtcaggctcagtttcccactatggcttacagcttaacgtgtttggtttgttgaatgttaacttggttttgtcaagctcagttttttactctggcttacagcataacatgtttgacttttggttttgctgctttgttattgggttctgggtagttcttgatgaatccaaaagatcatgtgcacagccatattatctatttaagcgatccaggttattactatgaaaggatgccttctagctaaggagtagttaggttttttcttcaaggttaaattttctcgatgctctagtgttcctgtgaccataatcataataattcctttgaaagctctatggtccctggaagcagggcatacaatgcaagacagcaacttgatcacatcaactgaagtatacagggttctcttaactcttggtgacttcggtttaatggaccggttgtactcgtgttctatccgtaaccgttgtgatgtcttgtgtgtttggttgcgggatagctgggaccacgacgtttccgtctaattctgatggatagctatagacggcactgagatggttatattataacctctgatcctgaactctacgagatcgtctcatccgtcattgccaccaaatacaccattaaatta

SEQ ID NO: 6 - DNA, 552 bp, Artificial Sequence
  derived from Streptomyces viridochromogenes
atgagccccgaaaggaggcccgtcgaaatcaggcccgccaccgccgccgacatggccgccgtctgcgacatcgtgaaccactacatcgaaaccagcaccgtcaactttaggaccgaaccccagaccccccaggaatggatcgacgacctggaaaggctgcaggacagatacccctggctggtcgccgaagtcgaaggcgtcgtcgccggcatagcctacgccggcccctggaaggccaggaacgcctacgactggaccgtcgaaagcaccgtctacgtcagccacaggcaccagaggctgggcctgggcagcaccctgtacacccacctgctgaagagcatggaagcccagggcttcaagagcgtcgtcgccgtcatcggcctgcccaacgaccccagcgtcaggctgcacgaagccctgggctacaccgccaggggcaccctgagggccgccggctacaagcacggcggctggcacgacgtcggcttctggcagagggacttcgaactgcccgccccccccaggcccgtcaggcccgtcacccagatttga

SEQ ID NO: 7 - DNA, 5552 bp, Artificial Sequence
  derived from Streptomyces viridochromogenes and Zea mays
ggaaaaccaaaacaacgaataagcaaactgcaggaaaagtatgcagtggaaaccaacccagattcggacgataggaaagtatcaagtgaatgatttgccaggaaaaggagaggggtaaaaaggggcgaagatttagaagatctaaagcacaagaaccagagattagattgaacaatagggaacttggagcatcctttttttcttcagggaaaaactgaaaatccaaaccatgttgagcaaaaccgagtgggattggaaaccaaaaaacccgagataaagaaactcgagaaaaagcatgaaatcgaaaccaacttcagtaaaacaaaaggaggacagaaaagaaagtcggaagctataaagaatacattaacattcagtgaaacagcatgctgtcttcttctttttttatgcacaacagagcatacatatataccttcccaggctgaggacttggcggaggagagccgcggataggttggcggtgcagacggtctggacgggcccgaagacggagacgaacagcgggcccttcctgcccaggcaccacgcttggaacgccaagcacgcgccaaccgcggccccgccgaggacgacgatccccgcgacaagcgtggcgtcgatcctgggcgaccccaagccgaggaacctcccttccaggacgagccgtaggacggcggtgagagaggcacccgtcgcggaggtggcgcagcacaaggtgagcagcgcggggaaggcggcgagcgtggcggcctgcaggacggtgacgagcgcgaagacggtgacgccggcgacgaggcagcagcagccgaggttccagtcgtaggaggaagccggaccaaaccgggcaatgcaacctgcagatgcactagacggaggtaacgaggaggaggagaaaacagagcaagagcaggcggagagaagatagagcaaaacacgagtgaggcacagcgtaagcactcggtagaagtctccagaggcgaggtgcgcacaggagaacagatgagtaaagtcagccaaggatgcacgatccaacggctacgaatttttggagtgacgtggataggctcaaaggcgccatttccatccggctttatagtattttaaaaaaattcattttcctccctctagtgtgtgcggaggcgtgagcccgtttaacggcgttgagaagtctaacggacaccaaccacaaccaggaaccagcgccggccgcgccgccgagtgaagcagactgcatacggcacggcgcggcatctctctggctgcctctcgagagttccgcccccaccttcccgcggtagcgtggtggtttcgctttccgctgtcggcatccggaagttgcgtggcagagtggacggagacgaggccgggtcctccagctcctctcaaacgtcacggcaccggcatccggcagccagcgcggtccttcccaaccactcgttcccaacccatcccccttcctcgcccgccgtcataaatagccagccccatccccagcttctttccccaacctcatcttctctccttttgctctgaacgcacacaccgcccggtctccgatctccgatccccgatcccctcgtcgatcctaggtacggcgaccatcctaccccccccccccccccctctctctctgccttctctagatcggcgatccgatccatgcttacttggttagggcctgctaactatgttcatgtttgcgttagatccgtgcatggacgcgatctgtacacaccagacgcgttctgattgctagctaactcgccagtacctgggaatcctgggatggctgtagccggccccgcacgcagacgggaccgatttcatgattctctatttttttctttgtttcgttgcctagggtttcgttcgatcgatccgcgttattctttatttccatatattctggtacgatgttgatacggttcgaccgtgctgcttacgttctgtgcgcttgtttgccgggtcatttttaccttgccttttttgtatggtttggttgtggcgatgtggtctggtcgggctgtcgttctagatcggagtagagtgctgtttcaaactgtctagcggatctattagatttggatctgcatgtgtgacatatatcttcgtagttaagatgatgcatctgtatgtgtgacatgcggatctattagatttggatctgtatgtgtgacatatatcttcgtagttgagatgatgcatctgtatgtgtgacatatatcttcgtagttaagattatgcatggaaatatcaatcctttagataaggacgggtatacttgttgctgtgggttttactggtacttcgatagatgcatatacatgatctaacatgcttagatacatgaagtaacatgctgctacggtttaataattcttgagttgatttttactggtacttagatagatgtatatacatgcttagatacatgaagtaacatgctcctacagttcctttaatcattattgagtacctatatattctaataaatcagtatgttttaaattattttgattttactggtacttagatagatgtatatatacatgctcaaacatgcttagatacatgaagtaacatgctgctacggtttagtcattattgagtgcctatatattctaataaatcagtatgttttaaattattttgattttactggtacttagatagatgtatatatacatgctcaaacatgcttagatacatgaagtaatatgctactacggtttaattgttcttgagtacctatatattctaataaatcagtatgttttaaattatttcgattttactggtacttagatagatgtatatatacatgcttagatacatgaagtaacatgctactacggtttaattgttcttgaatacctatatattctaataaatcagtatgttttaaattatttcgattttactggtacttagatagatgtatatatacatgctcgaacatgcttagatacatgaagtaacatgctacatatatattataataaatcagtatgtcttaaattattttgattttactggtacttagatagatgtatatacatgctcaaacatgcttagatacatgaagtaacatgctactacggtttaatcattattgagtacctatatattctaataaatcagtatgttttcaattgttttgattttactggtacttagatatatgtatatatacatgctcgaacatgcttagatacgtgaagtaacatgctactatggttaattgttcttgagtacctatatattctaataaatcagtatgttttaaattatttcgattttactggtacttagatagatgtatatatacatgctcgaacatgcttagatacatgaagtaacatgctactacggtttaatcgttcttgagtacctatatattctaataaatcagtatgtcttaaattatcttgattttactggtacttagatagatgtatatacatgcttagatacatgaagtaacatgctactatgatttaatcgttcttgagtacctatatattctaataaatcagtatgtttttaattattttgattttactggtacttagatagatgtatatatacatgctcgaacatgcttagatacatgaagtaacatgctactacggtttaatcattcttgagtacctatatattctaataaatcagtatgtttttaattattttgatattactggtacttaacatgtttagatacatcatatagcatgcacatgctgctactgtttaatcattcgtgaatacctatatattctaatatatcagtatgtcttctaattattatgattttgatgtacttgtatggtggcatatgctgcagctatgtgtagattttgaatacccagtgtgatgagcatgcatggcgccttcatagttcatatgctgtttatttcctttgagactgttcttttttgttgatagtcaccctgttgtttggtgattcttatccagatccagatcttcgagatcctaaaccatgagccccgaaaggaggcccgtcgaaatcaggcccgccaccgccgccgacatggccgccgtctgcgacatcgtgaaccactacatcgaaaccagcaccgtcaactttaggaccgaaccccagaccccccaggaatggatcgacgacctggaaaggctgcaggacagatacccctggctggtcgccgaagtcgaaggcgtcgtcgccggcatagcctacgccggcccctggaaggccaggaacgcctacgactggaccgtcgaaagcaccgtctacgtcagccacaggcaccagaggctgggcctgggcagcaccctgtacacccacctgctgaagagcatggaagcccagggcttcaagagcgtcgtcgccgtcatcggcctgcccaacgaccccagcgtcaggctgcacgaagccctgggctacaccgccaggggcaccctgagggccgccggctacaagcacggcggctggcacgacgtcggcttctggcagagggacttcgaactgcccgccccccccaggcccgtcaggcccgtcacccagatttgagccaaggttcaattaagctgctgctgtacctgggtatctgcgtcgtctggtgccctctggtgtacctctatatggatctcgtcgtctaataaacatctgtggtttgtgtgtcatcaatcgtggttgtggcttcgttggtttaatggacctgttgtgtcctctgtgttgtacccaaaactcttctgcagcagtatggcttgaatccttatgaagtttgatatttgaacttaaaagtctgctcattatgtttttttctggttatatctcctaattaactgcctgggatcaaatttgattcgctggtgtttattggacccctcccaggttcttgctttctaccgtttcttgctgaatgttaacttgattctgtcaggctcagtttcccactatggcttacagcttaacgtgtttggtttgttgaatgttaacttggttttgtcaagctcagttttttactctggcttacagcataacatgtttgacttttggttttgctgctttgttattgggttctgggtagttcttgatgaatccaaaagatcatgtgcacagccatattatctatttaagcgatccaggttattactatgaaaggatgccttctagctaaggagtagttaggttttttcttcaaggttaaattttctcgatgctctagtgttcctgtgaccataatcataataattcctttgaaagctctatggtccctggaagcagggcatacaatgcaagacagcaacttgatcacatcaactgaagtatacagggttctcttaactcttggtgacttcggtttaatggaccggttgtactcgtgttctatccgtaaccgttgtgatgtcttgtgtgtttggttgcgggatagctgggaccacgacgtttccgtctaattctgatggatagctatagacggcactgagatggttatattataacctctgatcctgaactctacgagatcgtctcatccgtcattgccaccaaatacaccattaaatta

SEQ ID NO: 8 - DNA, 5527 bp, Artificial Sequence
  derived from Streptomyces viridochromogenes and Zea mays
ggaaaaccaaaacaacgaataagcaaactgcaggaaaagtatgcagtggaaaccaacccagattcggacgataggaaagtatcaagtgaatgatttgccaggaaaaggagaggggtaaaaaggggcgaagatttagaagatctaaagcacaagaaccagagattagattgaacaatagggaacttggagcatcctttttttcttcagggaaaaactgaaaatccaaaccatgttgagcaaaaccgagtgggattggaaaccaaaaaacccgagataaagaaactcgagaaaaagcatgaaatcgaaaccaacttcagtaaaacaaaaggaggacagaaaagaaagtcggaagctataaagaatacattaacattcagtgaaacagcatgctgtcttcttctttttttatgcacaacagagcatacatatataccttcccaggctgaggacttggcggaggagagccgcggataggttggcggtgcagacggtctggacgggcccgaagacggagacgaacagcgggcccttcctgcccaggcaccacgcttggaacgccaagcacgcgccaaccgcggccccgccgaggacgacgatccccgcgacaagcgtggcgtcgatcctgggcgaccccaagccgaggaacctcccttccaggacgagccgtaggacggcggtgagagaggcacccgtcgcggaggtggcgcagcacaaggtgagcagcgcggggaaggcggcgagcgtggcggcctgcaggacggtgacgagcgcgaagacggtgacgccggcgacgaggcagcagcagccgaggttccagtcgtaggaggaagccggaccaaaccgggcaatgcaacctgcagatgcactagacggaggtaacgaggaggaggagaaaacagagcaagagcaggcggagagaagatagagcaaaacacgagtgaggcacagcgtaagcactcggtagaagtctccagaggcgaggtgcgcacaggagaacagatgagtaaagtcagccaaggatgcacgatccaacggctacgaatttttggagtgacgtggataggctcaaaggcgccatttccatccggctttatagtattttaaaaaaattcattttcctccctctagtgtgtgcggaggcgtgagcccgtttaacggcgttgagaagtctaacggacaccaaccacaaccaggaaccagcgccggccgcgccgccgagtgaagcagactgcatacggcacggcgcggcatctctctggctgcctctcgagagttccgcccccaccttcccgcggtagcgtggtggtttcgctttccgctgtcggcatccggaagttgcgtggcagagtggacggagacgaggccgggtcctccagctcctctcaaacgtcacggcaccggcatccggcagccagcgcggtccttcccaaccactcgttcccaacccatcccccttcctcgcccgccgtcataaatagccagccccatccccagcttctttccccaacctcatcttctctccttttgctctgaacgcacacaccgcccggtctccgatctccgatccccgatcccctcgtcgatcctaggtacggcgaccatcctaccccccccccccccccctctctctctgccttctctagatcggcgatccgatccatgcttacttggttagggcctgctaactatgttcatgtttgcgttagatccgtgcatggacgcgatctgtacacaccagacgcgttctgattgctagctaactcgccagtacctgggaatcctgggatggctgtagccggccccgcacgcagacgggaccgatttcatgattctctatttttttctttgtttcgttgcctagggtttcgttcgatcgatccgcgttattctttatttccatatattctggtacgatgttgatacggttcgaccgtgctgcttacgttctgtgcgcttgtttgccgggtcatttttaccttgccttttttgtatggtttggttgtggcgatgtggtctggtcgggctgtcgttctagatcggagtagagtgctgtttcaaactgtctagcggatctattagatttggatctgcatgtgtgacatatatcttcgtagttaagatgatgcatctgtatgtgtgacatgcggatctattagatttggatctgtatgtgtgacatatatcttcgtagttgagatgatgcatctgtatgtgtgacatatatcttcgtagttaagattatgcatggaaatatcaatcctttagataaggacgggtatacttgttgctgtgggttttactggtacttcgatagatgcatatacatgatctaacatgcttagatacatgaagtaacatgctgctacggtttaataattcttgagttgatttttactggtacttagatagatgtatatacatgcttagatacatgaagtaacatgctcctacagttcctttaatcattattgagtacctatatattctaataaatcagtatgttttaaattattttgattttactggtacttagatagatgtatatatacatgctcaaacatgcttagatacatgaagtaacatgctgctacggtttagtcattattgagtgcctatatattctaataaatcagtatgttttaaattattttgattttactggtacttagatagatgtatatatacatgctcaaacatgcttagatacatgaagtaatatgctactacggtttaattgttcttgagtacctatatattctaataaatcagtatgttttaaattatttcgattttactggtacttagatagatgtatatatacatgcttagatacatgaagtaacatgctactacggtttaattgttcttgaatacctatatattctaataaatcagtatgttttaaattatttcgattttactggtacttagatagatgtatatatacatgctcgaacatgcttagatacatgaagtaacatgctacatatatattataataaatcagtatgtcttaaattattttgattttactggtacttagatagatgtatatacatgctcaaacatgcttagatacatgaagtaacatgctactacggtttaatcattattgagtacctatatattctaataaatcagtatgttttcaattgttttgattttactggtacttagatatatgtatatatacatgctcgaacatgcttagatacgtgaagtaacatgctactatggttaattgttcttgagtacctatatattctaataaatcagtatgttttaaattatttcgattttactggtacttagatagatgtatatatacatgctcgaacatgcttagatacatgaagtaacatgctactacggtttaatcgttcttgagtacctatatattctaataaatcagtatgtcttaaattatcttgattttactggtacttagatagatgtatatacatgcttagatacatgaagtaacatgctactatgatttaatcgttcttgagtacctatatattctaataaatcagtatgtttttaattattttgattttactggtacttagatagatgtatatatacatgctcgaacatgcttagatacatgaagtaacatgctactacggtttaatcattcttgagtacctatatattctaataaatcagtatgtttttaattattttgatattactggtacttaacatgtttagatacatcatatagcatgcacatgctgctactgtttaatcattcgtgaatacctatatattctaatatatcagtatgtcttctaattattatgattttgatgtacttgtatggtggcatatgctgcagctatgtgtagattttgaatacccagtgtgatgagcatgcatggcgccttcatagttcatatgctgtttatttcctttgagactgttcttttttgttgatagtcaccctgttgtttggtgattcttatccagatgagccccgaaaggaggcccgtcgaaatcaggcccgccaccgccgccgacatggccgccgtctgcgacatcgtgaaccactacatcgaaaccagcaccgtcaactttaggaccgaaccccagaccccccaggaatggatcgacgacctggaaaggctgcaggacagatacccctggctggtcgccgaagtcgaaggcgtcgtcgccggcatagcctacgccggcccctggaaggccaggaacgcctacgactggaccgtcgaaagcaccgtctacgtcagccacaggcaccagaggctgggcctgggcagcaccctgtacacccacctgctgaagagcatggaagcccagggcttcaagagcgtcgtcgccgtcatcggcctgcccaacgaccccagcgtcaggctgcacgaagccctgggctacaccgccaggggcaccctgagggccgccggctacaagcacggcggctggcacgacgtcggcttctggcagagggacttcgaactgcccgccccccccaggcccgtcaggcccgtcacccagatttgagccaaggttcaattaagctgctgctgtacctgggtatctgcgtcgtctggtgccctctggtgtacctctatatggatctcgtcgtctaataaacatctgtggtttgtgtgtcatcaatcgtggttgtggcttcgttggtttaatggacctgttgtgtcctctgtgttgtacccaaaactcttctgcagcagtatggcttgaatccttatgaagtttgatatttgaacttaaaagtctgctcattatgtttttttctggttatatctcctaattaactgcctgggatcaaatttgattcgctggtgtttattggacccctcccaggttcttgctttctaccgtttcttgctgaatgttaacttgattctgtcaggctcagtttcccactatggcttacagcttaacgtgtttggtttgttgaatgttaacttggttttgtcaagctcagttttttactctggcttacagcataacatgtttgacttttggttttgctgctttgttattgggttctgggtagttcttgatgaatccaaaagatcatgtgcacagccatattatctatttaagcgatccaggttattactatgaaaggatgccttctagctaaggagtagttaggttttttcttcaaggttaaattttctcgatgctctagtgttcctgtgaccataatcataataattcctttgaaagctctatggtccctggaagcagggcatacaatgcaagacagcaacttgatcacatcaactgaagtatacagggttctcttaactcttggtgacttcggtttaatggaccggttgtactcgtgttctatccgtaaccgttgtgatgtcttgtgtgtttggttgcgggatagctgggaccacgacgtttccgtctaattctgatggatagctatagacggcactgagatggttatattataacctctgatcctgaactctacgagatcgtctcatccgtcattgccaccaaatacaccattaaatta

SEQ ID NO: 9 - DNA, 6067 bp, Artificial Sequence
  derived from Streptomyces viridochromogenes and Zea mays
agctgcttgtggggaccagacaaaaaaggaatggtgcagaattgttaggcgcacctaccaaaagcaactttgcctttattgcaaagataaagcagattcctctagtacaagtggggaacaaaataacgtggaaaagagctgtcctgacagcccactcactattgcgtttgacgaacgcagtgacgaccacaaaactcgagacttttcaacaaagggtattatccggaaacctcctcggattccattgcccagctatctgtcactttattgtgaagatagtggaaaaggaaggtggctcctacaaatgccatcattgcgataaaggaaaggctatcgttgaagatgcctctgccgacagtggtcccaaagatggacccccacccacgaggagcatcgtggaaaaagaagacgttccaaccacgtcttcaaagcaagtggattgatgtgatatctccactgacgtaagggttgacgaacaatcccactatccttctgcctaattagctaacggacccggaaaaccaaaacaacgaataagcaaactgcaggaaaagtatgcagtggaaaccaacccagattcggacgataggaaagtatcaagtgaatgatttgccaggaaaaggagaggggtaaaaaggggcgaagatttagaagatctaaagcacaagaaccagagattagattgaacaatagggaacttggagcatcctttttttcttcagggaaaaactgaaaatccaaaccatgttgagcaaaaccgagtgggattggaaaccaaaaaacccgagataaagaaactcgagaaaaagcatgaaatcgaaaccaacttcagtaaaacaaaaggaggacagaaaagaaagtcggaagctataaagaatacattaacattcagtgaaacagcatgctgtcttcttctttttttatgcacaacagagcatacatatataccttcccaggctgaggacttggcggaggagagccgcggataggttggcggtgcagacggtctggacgggcccgaagacggagacgaacagcgggcccttcctgcccaggcaccacgcttggaacgccaagcacgcgccaaccgcggccccgccgaggacgacgatccccgcgacaagcgtggcgtcgatcctgggcgaccccaagccgaggaacctcccttccaggacgagccgtaggacggcggtgagagaggcacccgtcgcggaggtggcgcagcacaaggtgagcagcgcggggaaggcggcgagcgtggcggcctgcaggacggtgacgagcgcgaagacggtgacgccggcgacgaggcagcagcagccgaggttccagtcgtaggaggaagccggaccaaaccgggcaatgcaacctgcagatgcactagacggaggtaacgaggaggaggagaaaacagagcaagagcaggcggagagaagatagagcaaaacacgagtgaggcacagcgtaagcactcggtagaagtctccagaggcgaggtgcgcacaggagaacagatgagtaaagtcagccaaggatgcacgatccaacggctacgaatttttggagtgacgtggataggctcaaaggcgccatttccatccggctttatagtattttaaaaaaattcattttcctccctctagtgtgtgcggaggcgtgagcccgtttaacggcgttgagaagtctaacggacaccaaccacaaccaggaaccagcgccggccgcgccgccgagtgaagcagactgcatacggcacggcgcggcatctctctggctgcctctcgagagttccgcccccaccttcccgcggtagcgtggtggtttcgctttccgctgtcggcatccggaagttgcgtggcagagtggacggagacgaggccgggtcctccagctcctctcaaacgtcacggcaccggcatccggcagccagcgcggtccttcccaaccactcgttcccaacccatcccccttcctcgcccgccgtcataaatagccagccccatccccagcttctttccccaacctcatcttctctccttttgctctgaacgcacacaccgcccggtctccgatctccgatccccgatcccctcgtcgatcctaggtacggcgaccatcctaccccccccccccccccctctctctctgccttctctagatcggcgatccgatccatgcttacttggttagggcctgctaactatgttcatgtttgcgttagatccgtgcatggacgcgatctgtacacaccagacgcgttctgattgctagctaactcgccagtacctgggaatcctgggatggctgtagccggccccgcacgcagacgggaccgatttcatgattctctatttttttctttgtttcgttgcctagggtttcgttcgatcgatccgcgttattctttatttccatatattctggtacgatgttgatacggttcgaccgtgctgcttacgttctgtgcgcttgtttgccgggtcatttttaccttgccttttttgtatggtttggttgtggcgatgtggtctggtcgggctgtcgttctagatcggagtagagtgctgtttcaaactgtctagcggatctattagatttggatctgcatgtgtgacatatatcttcgtagttaagatgatgcatctgtatgtgtgacatgcggatctattagatttggatctgtatgtgtgacatatatcttcgtagttgagatgatgcatctgtatgtgtgacatatatcttcgtagttaagattatgcatggaaatatcaatcctttagataaggacgggtatacttgttgctgtgggttttactggtacttcgatagatgcatatacatgatctaacatgcttagatacatgaagtaacatgctgctacggtttaataattcttgagttgatttttactggtacttagatagatgtatatacatgcttagatacatgaagtaacatgctcctacagttcctttaatcattattgagtacctatatattctaataaatcagtatgttttaaattattttgattttactggtacttagatagatgtatatatacatgctcaaacatgcttagatacatgaagtaacatgctgctacggtttagtcattattgagtgcctatatattctaataaatcagtatgttttaaattattttgattttactggtacttagatagatgtatatatacatgctcaaacatgcttagatacatgaagtaatatgctactacggtttaattgttcttgagtacctatatattctaataaatcagtatgttttaaattatttcgattttactggtacttagatagatgtatatatacatgcttagatacatgaagtaacatgctactacggtttaattgttcttgaatacctatatattctaataaatcagtatgttttaaattatttcgattttactggtacttagatagatgtatatatacatgctcgaacatgcttagatacatgaagtaacatgctacatatatattataataaatcagtatgtcttaaattattttgattttactggtacttagatagatgtatatacatgctcaaacatgcttagatacatgaagtaacatgctactacggtttaatcattattgagtacctatatattctaataaatcagtatgttttcaattgttttgattttactggtacttagatatatgtatatatacatgctcgaacatgcttagatacgtgaagtaacatgctactatggttaattgttcttgagtacctatatattctaataaatcagtatgttttaaattatttcgattttactggtacttagatagatgtatatatacatgctcgaacatgcttagatacatgaagtaacatgctactacggtttaatcgttcttgagtacctatatattctaataaatcagtatgtcttaaattatcttgattttactggtacttagatagatgtatatacatgcttagatacatgaagtaacatgctactatgatttaatcgttcttgagtacctatatattctaataaatcagtatgtttttaattattttgattttactggtacttagatagatgtatatatacatgctcgaacatgcttagatacatgaagtaacatgctactacggtttaatcattcttgagtacctatatattctaataaatcagtatgtttttaattattttgatattactggtacttaacatgtttagatacatcatatagcatgcacatgctgctactgtttaatcattcgtgaatacctatatattctaatatatcagtatgtcttctaattattatgattttgatgtacttgtatggtggcatatgctgcagctatgtgtagattttgaatacccagtgtgatgagcatgcatggcgccttcatagttcatatgctgtttatttcctttgagactgttcttttttgttgatagtcaccctgttgtttggtgattcttatccagatccagatcttcgagatcctaaaccatgagccccgaaaggaggcccgtcgaaatcaggcccgccaccgccgccgacatggccgccgtctgcgacatcgtgaaccactacatcgaaaccagcaccgtcaactttaggaccgaaccccagaccccccaggaatggatcgacgacctggaaaggctgcaggacagatacccctggctggtcgccgaagtcgaaggcgtcgtcgccggcatagcctacgccggcccctggaaggccaggaacgcctacgactggaccgtcgaaagcaccgtctacgtcagccacaggcaccagaggctgggcctgggcagcaccctgtacacccacctgctgaagagcatggaagcccagggcttcaagagcgtcgtcgccgtcatcggcctgcccaacgaccccagcgtcaggctgcacgaagccctgggctacaccgccaggggcaccctgagggccgccggctacaagcacggcggctggcacgacgtcggcttctggcagagggacttcgaactgcccgccccccccaggcccgtcaggcccgtcacccagatttgagccaaggttcaattaagctgctgctgtacctgggtatctgcgtcgtctggtgccctctggtgtacctctatatggatctcgtcgtctaataaacatctgtggtttgtgtgtcatcaatcgtggttgtggcttcgttggtttaatggacctgttgtgtcctctgtgttgtacccaaaactcttctgcagcagtatggcttgaatccttatgaagtttgatatttgaacttaaaagtctgctcattatgtttttttctggttatatctcctaattaactgcctgggatcaaatttgattcgctggtgtttattggacccctcccaggttcttgctttctaccgtttcttgctgaatgttaacttgattctgtcaggctcagtttcccactatggcttacagcttaacgtgtttggtttgttgaatgttaacttggttttgtcaagctcagttttttactctggcttacagcataacatgtttgacttttggttttgctgctttgttattgggttctgggtagttcttgatgaatccaaaagatcatgtgcacagccatattatctatttaagcgatccaggttattactatgaaaggatgccttctagctaaggagtagttaggttttttcttcaaggttaaattttctcgatgctctagtgttcctgtgaccataatcataataattcctttgaaagctctatggtccctggaagcagggcatacaatgcaagacagcaacttgatcacatcaactgaagtatacagggttctcttaactcttggtgacttcggtttaatggaccggttgtactcgtgttctatccgtaaccgttgtgatgtcttgtgtgtttggttgcgggatagctgggaccacgacgtttccgtctaattctgatggatagctatagacggcactgagatggttatattataacctctgatcctgaactctacgagatcgtctcatccgtcattgccaccaaatacaccattaaatta

SEQ ID NO: 10 - DNA, 6042 bp, Artificial Sequence
  derived from Streptomyces viridochromogenes and Zea mays
agctgcttgtggggaccagacaaaaaaggaatggtgcagaattgttaggcgcacctaccaaaagcaactttgcctttattgcaaagataaagcagattcctctagtacaagtggggaacaaaataacgtggaaaagagctgtcctgacagcccactcactattgcgtttgacgaacgcagtgacgaccacaaaactcgagacttttcaacaaagggtattatccggaaacctcctcggattccattgcccagctatctgtcactttattgtgaagatagtggaaaaggaaggtggctcctacaaatgccatcattgcgataaaggaaaggctatcgttgaagatgcctctgccgacagtggtcccaaagatggacccccacccacgaggagcatcgtggaaaaagaagacgttccaaccacgtcttcaaagcaagtggattgatgtgatatctccactgacgtaagggttgacgaacaatcccactatccttctgcctaattagctaacggacccggaaaaccaaaacaacgaataagcaaactgcaggaaaagtatgcagtggaaaccaacccagattcggacgataggaaagtatcaagtgaatgatttgccaggaaaaggagaggggtaaaaaggggcgaagatttagaagatctaaagcacaagaaccagagattagattgaacaatagggaacttggagcatcctttttttcttcagggaaaaactgaaaatccaaaccatgttgagcaaaaccgagtgggattggaaaccaaaaaacccgagataaagaaactcgagaaaaagcatgaaatcgaaaccaacttcagtaaaacaaaaggaggacagaaaagaaagtcggaagctataaagaatacattaacattcagtgaaacagcatgctgtcttcttctttttttatgcacaacagagcatacatatataccttcccaggctgaggacttggcggaggagagccgcggataggttggcggtgcagacggtctggacgggcccgaagacggagacgaacagcgggcccttcctgcccaggcaccacgcttggaacgccaagcacgcgccaaccgcggccccgccgaggacgacgatccccgcgacaagcgtggcgtcgatcctgggcgaccccaagccgaggaacctcccttccaggacgagccgtaggacggcggtgagagaggcacccgtcgcggaggtggcgcagcacaaggtgagcagcgcggggaaggcggcgagcgtggcggcctgcaggacggtgacgagcgcgaagacggtgacgccggcgacgaggcagcagcagccgaggttccagtcgtaggaggaagccggaccaaaccgggcaatgcaacctgcagatgcactagacggaggtaacgaggaggaggagaaaacagagcaagagcaggcggagagaagatagagcaaaacacgagtgaggcacagcgtaagcactcggtagaagtctccagaggcgaggtgcgcacaggagaacagatgagtaaagtcagccaaggatgcacgatccaacggctacgaatttttggagtgacgtggataggctcaaaggcgccatttccatccggctttatagtattttaaaaaaattcattttcctccctctagtgtgtgcggaggcgtgagcccgtttaacggcgttgagaagtctaacggacaccaaccacaaccaggaaccagcgccggccgcgccgccgagtgaagcagactgcatacggcacggcgcggcatctctctggctgcctctcgagagttccgcccccaccttcccgcggtagcgtggtggtttcgctttccgctgtcggcatccggaagttgcgtggcagagtggacggagacgaggccgggtcctccagctcctctcaaacgtcacggcaccggcatccggcagccagcgcggtccttcccaaccactcgttcccaacccatcccccttcctcgcccgccgtcataaatagccagccccatccccagcttctttccccaacctcatcttctctccttttgctctgaacgcacacaccgcccggtctccgatctccgatccccgatcccctcgtcgatcctaggtacggcgaccatcctaccccccccccccccccctctctctctgccttctctagatcggcgatccgatccatgcttacttggttagggcctgctaactatgttcatgtttgcgttagatccgtgcatggacgcgatctgtacacaccagacgcgttctgattgctagctaactcgccagtacctgggaatcctgggatggctgtagccggccccgcacgcagacgggaccgatttcatgattctctatttttttctttgtttcgttgcctagggtttcgttcgatcgatccgcgttattctttatttccatatattctggtacgatgttgatacggttcgaccgtgctgcttacgttctgtgcgcttgtttgccgggtcatttttaccttgccttttttgtatggtttggttgtggcgatgtggtctggtcgggctgtcgttctagatcggagtagagtgctgtttcaaactgtctagcggatctattagatttggatctgcatgtgtgacatatatcttcgtagttaagatgatgcatctgtatgtgtgacatgcggatctattagatttggatctgtatgtgtgacatatatcttcgtagttgagatgatgcatctgtatgtgtgacatatatcttcgtagttaagattatgcatggaaatatcaatcctttagataaggacgggtatacttgttgctgtgggttttactggtacttcgatagatgcatatacatgatctaacatgcttagatacatgaagtaacatgctgctacggtttaataattcttgagttgatttttactggtacttagatagatgtatatacatgcttagatacatgaagtaacatgctcctacagttcctttaatcattattgagtacctatatattctaataaatcagtatgttttaaattattttgattttactggtacttagatagatgtatatatacatgctcaaacatgcttagatacatgaagtaacatgctgctacggtttagtcattattgagtgcctatatattctaataaatcagtatgttttaaattattttgattttactggtacttagatagatgtatatatacatgctcaaacatgcttagatacatgaagtaatatgctactacggtttaattgttcttgagtacctatatattctaataaatcagtatgttttaaattatttcgattttactggtacttagatagatgtatatatacatgcttagatacatgaagtaacatgctactacggtttaattgttcttgaatacctatatattctaataaatcagtatgttttaaattatttcgattttactggtacttagatagatgtatatatacatgctcgaacatgcttagatacatgaagtaacatgctacatatatattataataaatcagtatgtcttaaattattttgattttactggtacttagatagatgtatatacatgctcaaacatgcttagatacatgaagtaacatgctactacggtttaatcattattgagtacctatatattctaataaatcagtatgttttcaattgttttgattttactggtacttagatatatgtatatatacatgctcgaacatgcttagatacgtgaagtaacatgctactatggttaattgttcttgagtacctatatattctaataaatcagtatgttttaaattatttcgattttactggtacttagatagatgtatatatacatgctcgaacatgcttagatacatgaagtaacatgctactacggtttaatcgttcttgagtacctatatattctaataaatcagtatgtcttaaattatcttgattttactggtacttagatagatgtatatacatgcttagatacatgaagtaacatgctactatgatttaatcgttcttgagtacctatatattctaataaatcagtatgtttttaattattttgattttactggtacttagatagatgtatatatacatgctcgaacatgcttagatacatgaagtaacatgctactacggtttaatcattcttgagtacctatatattctaataaatcagtatgtttttaattattttgatattactggtacttaacatgtttagatacatcatatagcatgcacatgctgctactgtttaatcattcgtgaatacctatatattctaatatatcagtatgtcttctaattattatgattttgatgtacttgtatggtggcatatgctgcagctatgtgtagattttgaatacccagtgtgatgagcatgcatggcgccttcatagttcatatgctgtttatttcctttgagactgttcttttttgttgatagtcaccctgttgtttggtgattcttatccagatgagccccgaaaggaggcccgtcgaaatcaggcccgccaccgccgccgacatggccgccgtctgcgacatcgtgaaccactacatcgaaaccagcaccgtcaactttaggaccgaaccccagaccccccaggaatggatcgacgacctggaaaggctgcaggacagatacccctggctggtcgccgaagtcgaaggcgtcgtcgccggcatagcctacgccggcccctggaaggccaggaacgcctacgactggaccgtcgaaagcaccgtctacgtcagccacaggcaccagaggctgggcctgggcagcaccctgtacacccacctgctgaagagcatggaagcccagggcttcaagagcgtcgtcgccgtcatcggcctgcccaacgaccccagcgtcaggctgcacgaagccctgggctacaccgccaggggcaccctgagggccgccggctacaagcacggcggctggcacgacgtcggcttctggcagagggacttcgaactgcccgccccccccaggcccgtcaggcccgtcacccagatttgagccaaggttcaattaagctgctgctgtacctgggtatctgcgtcgtctggtgccctctggtgtacctctatatggatctcgtcgtctaataaacatctgtggtttgtgtgtcatcaatcgtggttgtggcttcgttggtttaatggacctgttgtgtcctctgtgttgtacccaaaactcttctgcagcagtatggcttgaatccttatgaagtttgatatttgaacttaaaagtctgctcattatgtttttttctggttatatctcctaattaactgcctgggatcaaatttgattcgctggtgtttattggacccctcccaggttcttgctttctaccgtttcttgctgaatgttaacttgattctgtcaggctcagtttcccactatggcttacagcttaacgtgtttggtttgttgaatgttaacttggttttgtcaagctcagttttttactctggcttacagcataacatgtttgacttttggttttgctgctttgttattgggttctgggtagttcttgatgaatccaaaagatcatgtgcacagccatattatctatttaagcgatccaggttattactatgaaaggatgccttctagctaaggagtagttaggttttttcttcaaggttaaattttctcgatgctctagtgttcctgtgaccataatcataataattcctttgaaagctctatggtccctggaagcagggcatacaatgcaagacagcaacttgatcacatcaactgaagtatacagggttctcttaactcttggtgacttcggtttaatggaccggttgtactcgtgttctatccgtaaccgttgtgatgtcttgtgtgtttggttgcgggatagctgggaccacgacgtttccgtctaattctgatggatagctatagacggcactgagatggttatattataacctctgatcctgaactctacgagatcgtctcatccgtcattgccaccaaatacaccattaaatta

SEQ ID NO: 11 - DNA, 552 bp, Artificial Sequence
  derived from Streptomyces viridochromogenes
atgtccccagagcgccggccggtggagatcaggccagccaccgccgccgacatggccgccgtgtgcgacatcgtgaaccactacatcgagacctccaccgtgaacttccggaccgagccgcagaccccacaggagtggatcgacgacctcgagcggctccaggaccgatacccgtggctcgtggccgaggtggagggcgtggtggccggcatcgcctacgccggcccctggaaggctaggaacgcctacgactggaccgtggagtccaccgtgtacgtgtcccaccgccaccagaggctcggcctcggctccaccctctacacccacctcctcaagtctatggaggcccagggcttcaagtccgtggtggccgtgatcggcctaccgaacgacccatccgtgcggctccacgaggccctcggctacaccgcccgaggcacgctcagggccgccggctacaagcacggcggctggcacgacgtgggcttctggcagagggacttcgagctgccagccccgccaaggccagtgcggccggtgacccagatttga

SEQ ID NO: 12 - DNA, 5552 bp, Artificial Sequence
  derived from Streptomyces viridochromogenes and Zea mays
ggaaaaccaaaacaacgaataagcaaactgcaggaaaagtatgcagtggaaaccaacccagattcggacgataggaaagtatcaagtgaatgatttgccaggaaaaggagaggggtaaaaaggggcgaagatttagaagatctaaagcacaagaaccagagattagattgaacaatagggaacttggagcatcctttttttcttcagggaaaaactgaaaatccaaaccatgttgagcaaaaccgagtgggattggaaaccaaaaaacccgagataaagaaactcgagaaaaagcatgaaatcgaaaccaacttcagtaaaacaaaaggaggacagaaaagaaagtcggaagctataaagaatacattaacattcagtgaaacagcatgctgtcttcttctttttttatgcacaacagagcatacatatataccttcccaggctgaggacttggcggaggagagccgcggataggttggcggtgcagacggtctggacgggcccgaagacggagacgaacagcgggcccttcctgcccaggcaccacgcttggaacgccaagcacgcgccaaccgcggccccgccgaggacgacgatccccgcgacaagcgtggcgtcgatcctgggcgaccccaagccgaggaacctcccttccaggacgagccgtaggacggcggtgagagaggcacccgtcgcggaggtggcgcagcacaaggtgagcagcgcggggaaggcggcgagcgtggcggcctgcaggacggtgacgagcgcgaagacggtgacgccggcgacgaggcagcagcagccgaggttccagtcgtaggaggaagccggaccaaaccgggcaatgcaacctgcagatgcactagacggaggtaacgaggaggaggagaaaacagagcaagagcaggcggagagaagatagagcaaaacacgagtgaggcacagcgtaagcactcggtagaagtctccagaggcgaggtgcgcacaggagaacagatgagtaaagtcagccaaggatgcacgatccaacggctacgaatttttggagtgacgtggataggctcaaaggcgccatttccatccggctttatagtattttaaaaaaattcattttcctccctctagtgtgtgcggaggcgtgagcccgtttaacggcgttgagaagtctaacggacaccaaccacaaccaggaaccagcgccggccgcgccgccgagtgaagcagactgcatacggcacggcgcggcatctctctggctgcctctcgagagttccgcccccaccttcccgcggtagcgtggtggtttcgctttccgctgtcggcatccggaagttgcgtggcagagtggacggagacgaggccgggtcctccagctcctctcaaacgtcacggcaccggcatccggcagccagcgcggtccttcccaaccactcgttcccaacccatcccccttcctcgcccgccgtcataaatagccagccccatccccagcttctttccccaacctcatcttctctccttttgctctgaacgcacacaccgcccggtctccgatctccgatccccgatcccctcgtcgatcctaggtacggcgaccatcctaccccccccccccccccctctctctctgccttctctagatcggcgatccgatccatgcttacttggttagggcctgctaactatgttcatgtttgcgttagatccgtgcatggacgcgatctgtacacaccagacgcgttctgattgctagctaactcgccagtacctgggaatcctgggatggctgtagccggccccgcacgcagacgggaccgatttcatgattctctatttttttctttgtttcgttgcctagggtttcgttcgatcgatccgcgttattctttatttccatatattctggtacgatgttgatacggttcgaccgtgctgcttacgttctgtgcgcttgtttgccgggtcatttttaccttgccttttttgtatggtttggttgtggcgatgtggtctggtcgggctgtcgttctagatcggagtagagtgctgtttcaaactgtctagcggatctattagatttggatctgcatgtgtgacatatatcttcgtagttaagatgatgcatctgtatgtgtgacatgcggatctattagatttggatctgtatgtgtgacatatatcttcgtagttgagatgatgcatctgtatgtgtgacatatatcttcgtagttaagattatgcatggaaatatcaatcctttagataaggacgggtatacttgttgctgtgggttttactggtacttcgatagatgcatatacatgatctaacatgcttagatacatgaagtaacatgctgctacggtttaataattcttgagttgatttttactggtacttagatagatgtatatacatgcttagatacatgaagtaacatgctcctacagttcctttaatcattattgagtacctatatattctaataaatcagtatgttttaaattattttgattttactggtacttagatagatgtatatatacatgctcaaacatgcttagatacatgaagtaacatgctgctacggtttagtcattattgagtgcctatatattctaataaatcagtatgttttaaattattttgattttactggtacttagatagatgtatatatacatgctcaaacatgcttagatacatgaagtaatatgctactacggtttaattgttcttgagtacctatatattctaataaatcagtatgttttaaattatttcgattttactggtacttagatagatgtatatatacatgcttagatacatgaagtaacatgctactacggtttaattgttcttgaatacctatatattctaataaatcagtatgttttaaattatttcgattttactggtacttagatagatgtatatatacatgctcgaacatgcttagatacatgaagtaacatgctacatatatattataataaatcagtatgtcttaaattattttgattttactggtacttagatagatgtatatacatgctcaaacatgcttagatacatgaagtaacatgctactacggtttaatcattattgagtacctatatattctaataaatcagtatgttttcaattgttttgattttactggtacttagatatatgtatatatacatgctcgaacatgcttagatacgtgaagtaacatgctactatggttaattgttcttgagtacctatatattctaataaatcagtatgttttaaattatttcgattttactggtacttagatagatgtatatatacatgctcgaacatgcttagatacatgaagtaacatgctactacggtttaatcgttcttgagtacctatatattctaataaatcagtatgtcttaaattatcttgattttactggtacttagatagatgtatatacatgcttagatacatgaagtaacatgctactatgatttaatcgttcttgagtacctatatattctaataaatcagtatgtttttaattattttgattttactggtacttagatagatgtatatatacatgctcgaacatgcttagatacatgaagtaacatgctactacggtttaatcattcttgagtacctatatattctaataaatcagtatgtttttaattattttgatattactggtacttaacatgtttagatacatcatatagcatgcacatgctgctactgtttaatcattcgtgaatacctatatattctaatatatcagtatgtcttctaattattatgattttgatgtacttgtatggtggcatatgctgcagctatgtgtagattttgaatacccagtgtgatgagcatgcatggcgccttcatagttcatatgctgtttatttcctttgagactgttcttttttgttgatagtcaccctgttgtttggtgattcttatccagatccagatcttcgagatcctaaaccatgtccccagagcgccggccggtggagatcaggccagccaccgccgccgacatggccgccgtgtgcgacatcgtgaaccactacatcgagacctccaccgtgaacttccggaccgagccgcagaccccacaggagtggatcgacgacctcgagcggctccaggaccgatacccgtggctcgtggccgaggtggagggcgtggtggccggcatcgcctacgccggcccctggaaggctaggaacgcctacgactggaccgtggagtccaccgtgtacgtgtcccaccgccaccagaggctcggcctcggctccaccctctacacccacctcctcaagtctatggaggcccagggcttcaagtccgtggtggccgtgatcggcctaccgaacgacccatccgtgcggctccacgaggccctcggctacaccgcccgaggcacgctcagggccgccggctacaagcacggcggctggcacgacgtgggcttctggcagagggacttcgagctgccagccccgccaaggccagtgcggccggtgacccagatttgagccaaggttcaattaagctgctgctgtacctgggtatctgcgtcgtctggtgccctctggtgtacctctatatggatctcgtcgtctaataaacatctgtggtttgtgtgtcatcaatcgtggttgtggcttcgttggtttaatggacctgttgtgtcctctgtgttgtacccaaaactcttctgcagcagtatggcttgaatccttatgaagtttgatatttgaacttaaaagtctgctcattatgtttttttctggttatatctcctaattaactgcctgggatcaaatttgattcgctggtgtttattggacccctcccaggttcttgctttctaccgtttcttgctgaatgttaacttgattctgtcaggctcagtttcccactatggcttacagcttaacgtgtttggtttgttgaatgttaacttggttttgtcaagctcagttttttactctggcttacagcataacatgtttgacttttggttttgctgctttgttattgggttctgggtagttcttgatgaatccaaaagatcatgtgcacagccatattatctatttaagcgatccaggttattactatgaaaggatgccttctagctaaggagtagttaggttttttcttcaaggttaaattttctcgatgctctagtgttcctgtgaccataatcataataattcctttgaaagctctatggtccctggaagcagggcatacaatgcaagacagcaacttgatcacatcaactgaagtatacagggttctcttaactcttggtgacttcggtttaatggaccggttgtactcgtgttctatccgtaaccgttgtgatgtcttgtgtgtttggttgcgggatagctgggaccacgacgtttccgtctaattctgatggatagctatagacggcactgagatggttatattataacctctgatcctgaactctacgagatcgtctcatccgtcattgccaccaaatacaccattaaatta

SEQ ID NO: 13 - DNA, 5527 bp, Artificial Sequence
  derived from Streptomyces viridochromogenes and Zea mays
ggaaaaccaaaacaacgaataagcaaactgcaggaaaagtatgcagtggaaaccaacccagattcggacgataggaaagtatcaagtgaatgatttgccaggaaaaggagaggggtaaaaaggggcgaagatttagaagatctaaagcacaagaaccagagattagattgaacaatagggaacttggagcatcctttttttcttcagggaaaaactgaaaatccaaaccatgttgagcaaaaccgagtgggattggaaaccaaaaaacccgagataaagaaactcgagaaaaagcatgaaatcgaaaccaacttcagtaaaacaaaaggaggacagaaaagaaagtcggaagctataaagaatacattaacattcagtgaaacagcatgctgtcttcttctttttttatgcacaacagagcatacatatataccttcccaggctgaggacttggcggaggagagccgcggataggttggcggtgcagacggtctggacgggcccgaagacggagacgaacagcgggcccttcctgcccaggcaccacgcttggaacgccaagcacgcgccaaccgcggccccgccgaggacgacgatccccgcgacaagcgtggcgtcgatcctgggcgaccccaagccgaggaacctcccttccaggacgagccgtaggacggcggtgagagaggcacccgtcgcggaggtggcgcagcacaaggtgagcagcgcggggaaggcggcgagcgtggcggcctgcaggacggtgacgagcgcgaagacggtgacgccggcgacgaggcagcagcagccgaggttccagtcgtaggaggaagccggaccaaaccgggcaatgcaacctgcagatgcactagacggaggtaacgaggaggaggagaaaacagagcaagagcaggcggagagaagatagagcaaaacacgagtgaggcacagcgtaagcactcggtagaagtctccagaggcgaggtgcgcacaggagaacagatgagtaaagtcagccaaggatgcacgatccaacggctacgaatttttggagtgacgtggataggctcaaaggcgccatttccatccggctttatagtattttaaaaaaattcattttcctccctctagtgtgtgcggaggcgtgagcccgtttaacggcgttgagaagtctaacggacaccaaccacaaccaggaaccagcgccggccgcgccgccgagtgaagcagactgcatacggcacggcgcggcatctctctggctgcctctcgagagttccgcccccaccttcccgcggtagcgtggtggtttcgctttccgctgtcggcatccggaagttgcgtggcagagtggacggagacgaggccgggtcctccagctcctctcaaacgtcacggcaccggcatccggcagccagcgcggtccttcccaaccactcgttcccaacccatcccccttcctcgcccgccgtcataaatagccagccccatccccagcttctttccccaacctcatcttctctccttttgctctgaacgcacacaccgcccggtctccgatctccgatccccgatcccctcgtcgatcctaggtacggcgaccatcctaccccccccccccccccctctctctctgccttctctagatcggcgatccgatccatgcttacttggttagggcctgctaactatgttcatgtttgcgttagatccgtgcatggacgcgatctgtacacaccagacgcgttctgattgctagctaactcgccagtacctgggaatcctgggatggctgtagccggccccgcacgcagacgggaccgatttcatgattctctatttttttctttgtttcgttgcctagggtttcgttcgatcgatccgcgttattctttatttccatatattctggtacgatgttgatacggttcgaccgtgctgcttacgttctgtgcgcttgtttgccgggtcatttttaccttgccttttttgtatggtttggttgtggcgatgtggtctggtcgggctgtcgttctagatcggagtagagtgctgtttcaaactgtctagcggatctattagatttggatctgcatgtgtgacatatatcttcgtagttaagatgatgcatctgtatgtgtgacatgcggatctattagatttggatctgtatgtgtgacatatatcttcgtagttgagatgatgcatctgtatgtgtgacatatatcttcgtagttaagattatgcatggaaatatcaatcctttagataaggacgggtatacttgttgctgtgggttttactggtacttcgatagatgcatatacatgatctaacatgcttagatacatgaagtaacatgctgctacggtttaataattcttgagttgatttttactggtacttagatagatgtatatacatgcttagatacatgaagtaacatgctcctacagttcctttaatcattattgagtacctatatattctaataaatcagtatgttttaaattattttgattttactggtacttagatagatgtatatatacatgctcaaacatgcttagatacatgaagtaacatgctgctacggtttagtcattattgagtgcctatatattctaataaatcagtatgttttaaattattttgattttactggtacttagatagatgtatatatacatgctcaaacatgcttagatacatgaagtaatatgctactacggtttaattgttcttgagtacctatatattctaataaatcagtatgttttaaattatttcgattttactggtacttagatagatgtatatatacatgcttagatacatgaagtaacatgctactacggtttaattgttcttgaatacctatatattctaataaatcagtatgttttaaattatttcgattttactggtacttagatagatgtatatatacatgctcgaacatgcttagatacatgaagtaacatgctacatatatattataataaatcagtatgtcttaaattattttgattttactggtacttagatagatgtatatacatgctcaaacatgcttagatacatgaagtaacatgctactacggtttaatcattattgagtacctatatattctaataaatcagtatgttttcaattgttttgattttactggtacttagatatatgtatatatacatgctcgaacatgcttagatacgtgaagtaacatgctactatggttaattgttcttgagtacctatatattctaataaatcagtatgttttaaattatttcgattttactggtacttagatagatgtatatatacatgctcgaacatgcttagatacatgaagtaacatgctactacggtttaatcgttcttgagtacctatatattctaataaatcagtatgtcttaaattatcttgattttactggtacttagatagatgtatatacatgcttagatacatgaagtaacatgctactatgatttaatcgttcttgagtacctatatattctaataaatcagtatgtttttaattattttgattttactggtacttagatagatgtatatatacatgctcgaacatgcttagatacatgaagtaacatgctactacggtttaatcattcttgagtacctatatattctaataaatcagtatgtttttaattattttgatattactggtacttaacatgtttagatacatcatatagcatgcacatgctgctactgtttaatcattcgtgaatacctatatattctaatatatcagtatgtcttctaattattatgattttgatgtacttgtatggtggcatatgctgcagctatgtgtagattttgaatacccagtgtgatgagcatgcatggcgccttcatagttcatatgctgtttatttcctttgagactgttcttttttgttgatagtcaccctgttgtttggtgattcttatccagatgtccccagagcgccggccggtggagatcaggccagccaccgccgccgacatggccgccgtgtgcgacatcgtgaaccactacatcgagacctccaccgtgaacttccggaccgagccgcagaccccacaggagtggatcgacgacctcgagcggctccaggaccgatacccgtggctcgtggccgaggtggagggcgtggtggccggcatcgcctacgccggcccctggaaggctaggaacgcctacgactggaccgtggagtccaccgtgtacgtgtcccaccgccaccagaggctcggcctcggctccaccctctacacccacctcctcaagtctatggaggcccagggcttcaagtccgtggtggccgtgatcggcctaccgaacgacccatccgtgcggctccacgaggccctcggctacaccgcccgaggcacgctcagggccgccggctacaagcacggcggctggcacgacgtgggcttctggcagagggacttcgagctgccagccccgccaaggccagtgcggccggtgacccagatttgagccaaggttcaattaagctgctgctgtacctgggtatctgcgtcgtctggtgccctctggtgtacctctatatggatctcgtcgtctaataaacatctgtggtttgtgtgtcatcaatcgtggttgtggcttcgttggtttaatggacctgttgtgtcctctgtgttgtacccaaaactcttctgcagcagtatggcttgaatccttatgaagtttgatatttgaacttaaaagtctgctcattatgtttttttctggttatatctcctaattaactgcctgggatcaaatttgattcgctggtgtttattggacccctcccaggttcttgctttctaccgtttcttgctgaatgttaacttgattctgtcaggctcagtttcccactatggcttacagcttaacgtgtttggtttgttgaatgttaacttggttttgtcaagctcagttttttactctggcttacagcataacatgtttgacttttggttttgctgctttgttattgggttctgggtagttcttgatgaatccaaaagatcatgtgcacagccatattatctatttaagcgatccaggttattactatgaaaggatgccttctagctaaggagtagttaggttttttcttcaaggttaaattttctcgatgctctagtgttcctgtgaccataatcataataattcctttgaaagctctatggtccctggaagcagggcatacaatgcaagacagcaacttgatcacatcaactgaagtatacagggttctcttaactcttggtgacttcggtttaatggaccggttgtactcgtgttctatccgtaaccgttgtgatgtcttgtgtgtttggttgcgggatagctgggaccacgacgtttccgtctaattctgatggatagctatagacggcactgagatggttatattataacctctgatcctgaactctacgagatcgtctcatccgtcattgccaccaaatacaccattaaatta

SEQ ID NO: 14 - DNA, 6067 bp, Artificial Sequence
  derived from Streptomyces viridochromogenes and Zea mays
agctgcttgtggggaccagacaaaaaaggaatggtgcagaattgttaggcgcacctaccaaaagcaactttgcctttattgcaaagataaagcagattcctctagtacaagtggggaacaaaataacgtggaaaagagctgtcctgacagcccactcactattgcgtttgacgaacgcagtgacgaccacaaaactcgagacttttcaacaaagggtattatccggaaacctcctcggattccattgcccagctatctgtcactttattgtgaagatagtggaaaaggaaggtggctcctacaaatgccatcattgcgataaaggaaaggctatcgttgaagatgcctctgccgacagtggtcccaaagatggacccccacccacgaggagcatcgtggaaaaagaagacgttccaaccacgtcttcaaagcaagtggattgatgtgatatctccactgacgtaagggttgacgaacaatcccactatccttctgcctaattagctaacggacccggaaaaccaaaacaacgaataagcaaactgcaggaaaagtatgcagtggaaaccaacccagattcggacgataggaaagtatcaagtgaatgatttgccaggaaaaggagaggggtaaaaaggggcgaagatttagaagatctaaagcacaagaaccagagattagattgaacaatagggaacttggagcatcctttttttcttcagggaaaaactgaaaatccaaaccatgttgagcaaaaccgagtgggattggaaaccaaaaaacccgagataaagaaactcgagaaaaagcatgaaatcgaaaccaacttcagtaaaacaaaaggaggacagaaaagaaagtcggaagctataaagaatacattaacattcagtgaaacagcatgctgtcttcttctttttttatgcacaacagagcatacatatataccttcccaggctgaggacttggcggaggagagccgcggataggttggcggtgcagacggtctggacgggcccgaagacggagacgaacagcgggcccttcctgcccaggcaccacgcttggaacgccaagcacgcgccaaccgcggccccgccgaggacgacgatccccgcgacaagcgtggcgtcgatcctgggcgaccccaagccgaggaacctcccttccaggacgagccgtaggacggcggtgagagaggcacccgtcgcggaggtggcgcagcacaaggtgagcagcgcggggaaggcggcgagcgtggcggcctgcaggacggtgacgagcgcgaagacggtgacgccggcgacgaggcagcagcagccgaggttccagtcgtaggaggaagccggaccaaaccgggcaatgcaacctgcagatgcactagacggaggtaacgaggaggaggagaaaacagagcaagagcaggcggagagaagatagagcaaaacacgagtgaggcacagcgtaagcactcggtagaagtctccagaggcgaggtgcgcacaggagaacagatgagtaaagtcagccaaggatgcacgatccaacggctacgaatttttggagtgacgtggataggctcaaaggcgccatttccatccggctttatagtattttaaaaaaattcattttcctccctctagtgtgtgcggaggcgtgagcccgtttaacggcgttgagaagtctaacggacaccaaccacaaccaggaaccagcgccggccgcgccgccgagtgaagcagactgcatacggcacggcgcggcatctctctggctgcctctcgagagttccgcccccaccttcccgcggtagcgtggtggtttcgctttccgctgtcggcatccggaagttgcgtggcagagtggacggagacgaggccgggtcctccagctcctctcaaacgtcacggcaccggcatccggcagccagcgcggtccttcccaaccactcgttcccaacccatcccccttcctcgcccgccgtcataaatagccagccccatccccagcttctttccccaacctcatcttctctccttttgctctgaacgcacacaccgcccggtctccgatctccgatccccgatcccctcgtcgatcctaggtacggcgaccatcctaccccccccccccccccctctctctctgccttctctagatcggcgatccgatccatgcttacttggttagggcctgctaactatgttcatgtttgcgttagatccgtgcatggacgcgatctgtacacaccagacgcgttctgattgctagctaactcgccagtacctgggaatcctgggatggctgtagccggccccgcacgcagacgggaccgatttcatgattctctatttttttctttgtttcgttgcctagggtttcgttcgatcgatccgcgttattctttatttccatatattctggtacgatgttgatacggttcgaccgtgctgcttacgttctgtgcgcttgtttgccgggtcatttttaccttgccttttttgtatggtttggttgtggcgatgtggtctggtcgggctgtcgttctagatcggagtagagtgctgtttcaaactgtctagcggatctattagatttggatctgcatgtgtgacatatatcttcgtagttaagatgatgcatctgtatgtgtgacatgcggatctattagatttggatctgtatgtgtgacatatatcttcgtagttgagatgatgcatctgtatgtgtgacatatatcttcgtagttaagattatgcatggaaatatcaatcctttagataaggacgggtatacttgttgctgtgggttttactggtacttcgatagatgcatatacatgatctaacatgcttagatacatgaagtaacatgctgctacggtttaataattcttgagttgatttttactggtacttagatagatgtatatacatgcttagatacatgaagtaacatgctcctacagttcctttaatcattattgagtacctatatattctaataaatcagtatgttttaaattattttgattttactggtacttagatagatgtatatatacatgctcaaacatgcttagatacatgaagtaacatgctgctacggtttagtcattattgagtgcctatatattctaataaatcagtatgttttaaattattttgattttactggtacttagatagatgtatatatacatgctcaaacatgcttagatacatgaagtaatatgctactacggtttaattgttcttgagtacctatatattctaataaatcagtatgttttaaattatttcgattttactggtacttagatagatgtatatatacatgcttagatacatgaagtaacatgctactacggtttaattgttcttgaatacctatatattctaataaatcagtatgttttaaattatttcgattttactggtacttagatagatgtatatatacatgctcgaacatgcttagatacatgaagtaacatgctacatatatattataataaatcagtatgtcttaaattattttgattttactggtacttagatagatgtatatacatgctcaaacatgcttagatacatgaagtaacatgctactacggtttaatcattattgagtacctatatattctaataaatcagtatgttttcaattgttttgattttactggtacttagatatatgtatatatacatgctcgaacatgcttagatacgtgaagtaacatgctactatggttaattgttcttgagtacctatatattctaataaatcagtatgttttaaattatttcgattttactggtacttagatagatgtatatatacatgctcgaacatgcttagatacatgaagtaacatgctactacggtttaatcgttcttgagtacctatatattctaataaatcagtatgtcttaaattatcttgattttactggtacttagatagatgtatatacatgcttagatacatgaagtaacatgctactatgatttaatcgttcttgagtacctatatattctaataaatcagtatgtttttaattattttgattttactggtacttagatagatgtatatatacatgctcgaacatgcttagatacatgaagtaacatgctactacggtttaatcattcttgagtacctatatattctaataaatcagtatgtttttaattattttgatattactggtacttaacatgtttagatacatcatatagcatgcacatgctgctactgtttaatcattcgtgaatacctatatattctaatatatcagtatgtcttctaattattatgattttgatgtacttgtatggtggcatatgctgcagctatgtgtagattttgaatacccagtgtgatgagcatgcatggcgccttcatagttcatatgctgtttatttcctttgagactgttcttttttgttgatagtcaccctgttgtttggtgattcttatccagatccagatcttcgagatcctaaaccatgtccccagagcgccggccggtggagatcaggccagccaccgccgccgacatggccgccgtgtgcgacatcgtgaaccactacatcgagacctccaccgtgaacttccggaccgagccgcagaccccacaggagtggatcgacgacctcgagcggctccaggaccgatacccgtggctcgtggccgaggtggagggcgtggtggccggcatcgcctacgccggcccctggaaggctaggaacgcctacgactggaccgtggagtccaccgtgtacgtgtcccaccgccaccagaggctcggcctcggctccaccctctacacccacctcctcaagtctatggaggcccagggcttcaagtccgtggtggccgtgatcggcctaccgaacgacccatccgtgcggctccacgaggccctcggctacaccgcccgaggcacgctcagggccgccggctacaagcacggcggctggcacgacgtgggcttctggcagagggacttcgagctgccagccccgccaaggccagtgcggccggtgacccagatttgagccaaggttcaattaagctgctgctgtacctgggtatctgcgtcgtctggtgccctctggtgtacctctatatggatctcgtcgtctaataaacatctgtggtttgtgtgtcatcaatcgtggttgtggcttcgttggtttaatggacctgttgtgtcctctgtgttgtacccaaaactcttctgcagcagtatggcttgaatccttatgaagtttgatatttgaacttaaaagtctgctcattatgtttttttctggttatatctcctaattaactgcctgggatcaaatttgattcgctggtgtttattggacccctcccaggttcttgctttctaccgtttcttgctgaatgttaacttgattctgtcaggctcagtttcccactatggcttacagcttaacgtgtttggtttgttgaatgttaacttggttttgtcaagctcagttttttactctggcttacagcataacatgtttgacttttggttttgctgctttgttattgggttctgggtagttcttgatgaatccaaaagatcatgtgcacagccatattatctatttaagcgatccaggttattactatgaaaggatgccttctagctaaggagtagttaggttttttcttcaaggttaaattttctcgatgctctagtgttcctgtgaccataatcataataattcctttgaaagctctatggtccctggaagcagggcatacaatgcaagacagcaacttgatcacatcaactgaagtatacagggttctcttaactcttggtgacttcggtttaatggaccggttgtactcgtgttctatccgtaaccgttgtgatgtcttgtgtgtttggttgcgggatagctgggaccacgacgtttccgtctaattctgatggatagctatagacggcactgagatggttatattataacctctgatcctgaactctacgagatcgtctcatccgtcattgccaccaaatacaccattaaatta

SEQ ID NO: 15 - DNA, 6042 bp, Artificial Sequence
  derived from Streptomyces viridochromogenes and Zea mays
agctgcttgtggggaccagacaaaaaaggaatggtgcagaattgttaggcgcacctaccaaaagcaactttgcctttattgcaaagataaagcagattcctctagtacaagtggggaacaaaataacgtggaaaagagctgtcctgacagcccactcactattgcgtttgacgaacgcagtgacgaccacaaaactcgagacttttcaacaaagggtattatccggaaacctcctcggattccattgcccagctatctgtcactttattgtgaagatagtggaaaaggaaggtggctcctacaaatgccatcattgcgataaaggaaaggctatcgttgaagatgcctctgccgacagtggtcccaaagatggacccccacccacgaggagcatcgtggaaaaagaagacgttccaaccacgtcttcaaagcaagtggattgatgtgatatctccactgacgtaagggttgacgaacaatcccactatccttctgcctaattagctaacggacccggaaaaccaaaacaacgaataagcaaactgcaggaaaagtatgcagtggaaaccaacccagattcggacgataggaaagtatcaagtgaatgatttgccaggaaaaggagaggggtaaaaaggggcgaagatttagaagatctaaagcacaagaaccagagattagattgaacaatagggaacttggagcatcctttttttcttcagggaaaaactgaaaatccaaaccatgttgagcaaaaccgagtgggattggaaaccaaaaaacccgagataaagaaactcgagaaaaagcatgaaatcgaaaccaacttcagtaaaacaaaaggaggacagaaaagaaagtcggaagctataaagaatacattaacattcagtgaaacagcatgctgtcttcttctttttttatgcacaacagagcatacatatataccttcccaggctgaggacttggcggaggagagccgcggataggttggcggtgcagacggtctggacgggcccgaagacggagacgaacagcgggcccttcctgcccaggcaccacgcttggaacgccaagcacgcgccaaccgcggccccgccgaggacgacgatccccgcgacaagcgtggcgtcgatcctgggcgaccccaagccgaggaacctcccttccaggacgagccgtaggacggcggtgagagaggcacccgtcgcggaggtggcgcagcacaaggtgagcagcgcggggaaggcggcgagcgtggcggcctgcaggacggtgacgagcgcgaagacggtgacgccggcgacgaggcagcagcagccgaggttccagtcgtaggaggaagccggaccaaaccgggcaatgcaacctgcagatgcactagacggaggtaacgaggaggaggagaaaacagagcaagagcaggcggagagaagatagagcaaaacacgagtgaggcacagcgtaagcactcggtagaagtctccagaggcgaggtgcgcacaggagaacagatgagtaaagtcagccaaggatgcacgatccaacggctacgaatttttggagtgacgtggataggctcaaaggcgccatttccatccggctttatagtattttaaaaaaattcattttcctccctctagtgtgtgcggaggcgtgagcccgtttaacggcgttgagaagtctaacggacaccaaccacaaccaggaaccagcgccggccgcgccgccgagtgaagcagactgcatacggcacggcgcggcatctctctggctgcctctcgagagttccgcccccaccttcccgcggtagcgtggtggtttcgctttccgctgtcggcatccggaagttgcgtggcagagtggacggagacgaggccgggtcctccagctcctctcaaacgtcacggcaccggcatccggcagccagcgcggtccttcccaaccactcgttcccaacccatcccccttcctcgcccgccgtcataaatagccagccccatccccagcttctttccccaacctcatcttctctccttttgctctgaacgcacacaccgcccggtctccgatctccgatccccgatcccctcgtcgatcctaggtacggcgaccatcctaccccccccccccccccctctctctctgccttctctagatcggcgatccgatccatgcttacttggttagggcctgctaactatgttcatgtttgcgttagatccgtgcatggacgcgatctgtacacaccagacgcgttctgattgctagctaactcgccagtacctgggaatcctgggatggctgtagccggccccgcacgcagacgggaccgatttcatgattctctatttttttctttgtttcgttgcctagggtttcgttcgatcgatccgcgttattctttatttccatatattctggtacgatgttgatacggttcgaccgtgctgcttacgttctgtgcgcttgtttgccgggtcatttttaccttgccttttttgtatggtttggttgtggcgatgtggtctggtcgggctgtcgttctagatcggagtagagtgctgtttcaaactgtctagcggatctattagatttggatctgcatgtgtgacatatatcttcgtagttaagatgatgcatctgtatgtgtgacatgcggatctattagatttggatctgtatgtgtgacatatatcttcgtagttgagatgatgcatctgtatgtgtgacatatatcttcgtagttaagattatgcatggaaatatcaatcctttagataaggacgggtatacttgttgctgtgggttttactggtacttcgatagatgcatatacatgatctaacatgcttagatacatgaagtaacatgctgctacggtttaataattcttgagttgatttttactggtacttagatagatgtatatacatgcttagatacatgaagtaacatgctcctacagttcctttaatcattattgagtacctatatattctaataaatcagtatgttttaaattattttgattttactggtacttagatagatgtatatatacatgctcaaacatgcttagatacatgaagtaacatgctgctacggtttagtcattattgagtgcctatatattctaataaatcagtatgttttaaattattttgattttactggtacttagatagatgtatatatacatgctcaaacatgcttagatacatgaagtaatatgctactacggtttaattgttcttgagtacctatatattctaataaatcagtatgttttaaattatttcgattttactggtacttagatagatgtatatatacatgcttagatacatgaagtaacatgctactacggtttaattgttcttgaatacctatatattctaataaatcagtatgttttaaattatttcgattttactggtacttagatagatgtatatatacatgctcgaacatgcttagatacatgaagtaacatgctacatatatattataataaatcagtatgtcttaaattattttgattttactggtacttagatagatgtatatacatgctcaaacatgcttagatacatgaagtaacatgctactacggtttaatcattattgagtacctatatattctaataaatcagtatgttttcaattgttttgattttactggtacttagatatatgtatatatacatgctcgaacatgcttagatacgtgaagtaacatgctactatggttaattgttcttgagtacctatatattctaataaatcagtatgttttaaattatttcgattttactggtacttagatagatgtatatatacatgctcgaacatgcttagatacatgaagtaacatgctactacggtttaatcgttcttgagtacctatatattctaataaatcagtatgtcttaaattatcttgattttactggtacttagatagatgtatatacatgcttagatacatgaagtaacatgctactatgatttaatcgttcttgagtacctatatattctaataaatcagtatgtttttaattattttgattttactggtacttagatagatgtatatatacatgctcgaacatgcttagatacatgaagtaacatgctactacggtttaatcattcttgagtacctatatattctaataaatcagtatgtttttaattattttgatattactggtacttaacatgtttagatacatcatatagcatgcacatgctgctactgtttaatcattcgtgaatacctatatattctaatatatcagtatgtcttctaattattatgattttgatgtacttgtatggtggcatatgctgcagctatgtgtagattttgaatacccagtgtgatgagcatgcatggcgccttcatagttcatatgctgtttatttcctttgagactgttcttttttgttgatagtcaccctgttgtttggtgattcttatccagatgtccccagagcgccggccggtggagatcaggccagccaccgccgccgacatggccgccgtgtgcgacatcgtgaaccactacatcgagacctccaccgtgaacttccggaccgagccgcagaccccacaggagtggatcgacgacctcgagcggctccaggaccgatacccgtggctcgtggccgaggtggagggcgtggtggccggcatcgcctacgccggcccctggaaggctaggaacgcctacgactggaccgtggagtccaccgtgtacgtgtcccaccgccaccagaggctcggcctcggctccaccctctacacccacctcctcaagtctatggaggcccagggcttcaagtccgtggtggccgtgatcggcctaccgaacgacccatccgtgcggctccacgaggccctcggctacaccgcccgaggcacgctcagggccgccggctacaagcacggcggctggcacgacgtgggcttctggcagagggacttcgagctgccagccccgccaaggccagtgcggccggtgacccagatttgagccaaggttcaattaagctgctgctgtacctgggtatctgcgtcgtctggtgccctctggtgtacctctatatggatctcgtcgtctaataaacatctgtggtttgtgtgtcatcaatcgtggttgtggcttcgttggtttaatggacctgttgtgtcctctgtgttgtacccaaaactcttctgcagcagtatggcttgaatccttatgaagtttgatatttgaacttaaaagtctgctcattatgtttttttctggttatatctcctaattaactgcctgggatcaaatttgattcgctggtgtttattggacccctcccaggttcttgctttctaccgtttcttgctgaatgttaacttgattctgtcaggctcagtttcccactatggcttacagcttaacgtgtttggtttgttgaatgttaacttggttttgtcaagctcagttttttactctggcttacagcataacatgtttgacttttggttttgctgctttgttattgggttctgggtagttcttgatgaatccaaaagatcatgtgcacagccatattatctatttaagcgatccaggttattactatgaaaggatgccttctagctaaggagtagttaggttttttcttcaaggttaaattttctcgatgctctagtgttcctgtgaccataatcataataattcctttgaaagctctatggtccctggaagcagggcatacaatgcaagacagcaacttgatcacatcaactgaagtatacagggttctcttaactcttggtgacttcggtttaatggaccggttgtactcgtgttctatccgtaaccgttgtgatgtcttgtgtgtttggttgcgggatagctgggaccacgacgtttccgtctaattctgatggatagctatagacggcactgagatggttatattataacctctgatcctgaactctacgagatcgtctcatccgtcattgccaccaaatacaccattaaatta

SEQ ID NO: 16 - DNA, 552 bp, Artificial Sequence
  derived from Streptomyces viridochromogenes
atgtccccagagaggaggccagtggagatcaggccagccaccgccgccgacatggccgccgtgtgcgacatcgtgaaccactacatcgagacctccaccgtgaacttcaggaccgagccacagaccccacaggagtggatcgacgacctcgagaggctccaggacagatacccctggctcgtggccgaggtggagggcgtggtggccggcatcgcctacgccggcccctggaaagctaggaacgcctacgactggaccgtggagtccaccgtgtacgtgtcccacaggcaccagaggctcggcctcggctccaccctctacacccacctcctcaagtctatggaggcccagggcttcaagtccgtggtggccgtgatcggcctaccaaacgacccatccgtgaggctccacgaggccctcggctacaccgcgagaggcaccctcagggccgccggctacaagcacggcggctggcacgacgtgggcttctggcagagggacttcgagctgccagccccaccaaggccagtgaggccagtgacccagatttga

SEQ ID NO: 17 - DNA, 5552 bp, Artificial Sequence
  derived from Streptomyces viridochromogenes and Zea mays
ggaaaaccaaaacaacgaataagcaaactgcaggaaaagtatgcagtggaaaccaacccagattcggacgataggaaagtatcaagtgaatgatttgccaggaaaaggagaggggtaaaaaggggcgaagatttagaagatctaaagcacaagaaccagagattagattgaacaatagggaacttggagcatcctttttttcttcagggaaaaactgaaaatccaaaccatgttgagcaaaaccgagtgggattggaaaccaaaaaacccgagataaagaaactcgagaaaaagcatgaaatcgaaaccaacttcagtaaaacaaaaggaggacagaaaagaaagtcggaagctataaagaatacattaacattcagtgaaacagcatgctgtcttcttctttttttatgcacaacagagcatacatatataccttcccaggctgaggacttggcggaggagagccgcggataggttggcggtgcagacggtctggacgggcccgaagacggagacgaacagcgggcccttcctgcccaggcaccacgcttggaacgccaagcacgcgccaaccgcggccccgccgaggacgacgatccccgcgacaagcgtggcgtcgatcctgggcgaccccaagccgaggaacctcccttccaggacgagccgtaggacggcggtgagagaggcacccgtcgcggaggtggcgcagcacaaggtgagcagcgcggggaaggcggcgagcgtggcggcctgcaggacggtgacgagcgcgaagacggtgacgccggcgacgaggcagcagcagccgaggttccagtcgtaggaggaagccggaccaaaccgggcaatgcaacctgcagatgcactagacggaggtaacgaggaggaggagaaaacagagcaagagcaggcggagagaagatagagcaaaacacgagtgaggcacagcgtaagcactcggtagaagtctccagaggcgaggtgcgcacaggagaacagatgagtaaagtcagccaaggatgcacgatccaacggctacgaatttttggagtgacgtggataggctcaaaggcgccatttccatccggctttatagtattttaaaaaaattcattttcctccctctagtgtgtgcggaggcgtgagcccgtttaacggcgttgagaagtctaacggacaccaaccacaaccaggaaccagcgccggccgcgccgccgagtgaagcagactgcatacggcacggcgcggcatctctctggctgcctctcgagagttccgcccccaccttcccgcggtagcgtggtggtttcgctttccgctgtcggcatccggaagttgcgtggcagagtggacggagacgaggccgggtcctccagctcctctcaaacgtcacggcaccggcatccggcagccagcgcggtccttcccaaccactcgttcccaacccatcccccttcctcgcccgccgtcataaatagccagccccatccccagcttctttccccaacctcatcttctctccttttgctctgaacgcacacaccgcccggtctccgatctccgatccccgatcccctcgtcgatcctaggtacggcgaccatcctaccccccccccccccccctctctctctgccttctctagatcggcgatccgatccatgcttacttggttagggcctgctaactatgttcatgtttgcgttagatccgtgcatggacgcgatctgtacacaccagacgcgttctgattgctagctaactcgccagtacctgggaatcctgggatggctgtagccggccccgcacgcagacgggaccgatttcatgattctctatttttttctttgtttcgttgcctagggtttcgttcgatcgatccgcgttattctttatttccatatattctggtacgatgttgatacggttcgaccgtgctgcttacgttctgtgcgcttgtttgccgggtcatttttaccttgccttttttgtatggtttggttgtggcgatgtggtctggtcgggctgtcgttctagatcggagtagagtgctgtttcaaactgtctagcggatctattagatttggatctgcatgtgtgacatatatcttcgtagttaagatgatgcatctgtatgtgtgacatgcggatctattagatttggatctgtatgtgtgacatatatcttcgtagttgagatgatgcatctgtatgtgtgacatatatcttcgtagttaagattatgcatggaaatatcaatcctttagataaggacgggtatacttgttgctgtgggttttactggtacttcgatagatgcatatacatgatctaacatgcttagatacatgaagtaacatgctgctacggtttaataattcttgagttgatttttactggtacttagatagatgtatatacatgcttagatacatgaagtaacatgctcctacagttcctttaatcattattgagtacctatatattctaataaatcagtatgttttaaattattttgattttactggtacttagatagatgtatatatacatgctcaaacatgcttagatacatgaagtaacatgctgctacggtttagtcattattgagtgcctatatattctaataaatcagtatgttttaaattattttgattttactggtacttagatagatgtatatatacatgctcaaacatgcttagatacatgaagtaatatgctactacggtttaattgttcttgagtacctatatattctaataaatcagtatgttttaaattatttcgattttactggtacttagatagatgtatatatacatgcttagatacatgaagtaacatgctactacggtttaattgttcttgaatacctatatattctaataaatcagtatgttttaaattatttcgattttactggtacttagatagatgtatatatacatgctcgaacatgcttagatacatgaagtaacatgctacatatatattataataaatcagtatgtcttaaattattttgattttactggtacttagatagatgtatatacatgctcaaacatgcttagatacatgaagtaacatgctactacggtttaatcattattgagtacctatatattctaataaatcagtatgttttcaattgttttgattttactggtacttagatatatgtatatatacatgctcgaacatgcttagatacgtgaagtaacatgctactatggttaattgttcttgagtacctatatattctaataaatcagtatgttttaaattatttcgattttactggtacttagatagatgtatatatacatgctcgaacatgcttagatacatgaagtaacatgctactacggtttaatcgttcttgagtacctatatattctaataaatcagtatgtcttaaattatcttgattttactggtacttagatagatgtatatacatgcttagatacatgaagtaacatgctactatgatttaatcgttcttgagtacctatatattctaataaatcagtatgtttttaattattttgattttactggtacttagatagatgtatatatacatgctcgaacatgcttagatacatgaagtaacatgctactacggtttaatcattcttgagtacctatatattctaataaatcagtatgtttttaattattttgatattactggtacttaacatgtttagatacatcatatagcatgcacatgctgctactgtttaatcattcgtgaatacctatatattctaatatatcagtatgtcttctaattattatgattttgatgtacttgtatggtggcatatgctgcagctatgtgtagattttgaatacccagtgtgatgagcatgcatggcgccttcatagttcatatgctgtttatttcctttgagactgttcttttttgttgatagtcaccctgttgtttggtgattcttatccagatccagatcttcgagatcctaaaccatgtccccagagaggaggccagtggagatcaggccagccaccgccgccgacatggccgccgtgtgcgacatcgtgaaccactacatcgagacctccaccgtgaacttcaggaccgagccacagaccccacaggagtggatcgacgacctcgagaggctccaggacagatacccctggctcgtggccgaggtggagggcgtggtggccggcatcgcctacgccggcccctggaaagctaggaacgcctacgactggaccgtggagtccaccgtgtacgtgtcccacaggcaccagaggctcggcctcggctccaccctctacacccacctcctcaagtctatggaggcccagggcttcaagtccgtggtggccgtgatcggcctaccaaacgacccatccgtgaggctccacgaggccctcggctacaccgcgagaggcaccctcagggccgccggctacaagcacggcggctggcacgacgtgggcttctggcagagggacttcgagctgccagccccaccaaggccagtgaggccagtgacccagatttgagccaaggttcaattaagctgctgctgtacctgggtatctgcgtcgtctggtgccctctggtgtacctctatatggatctcgtcgtctaataaacatctgtggtttgtgtgtcatcaatcgtggttgtggcttcgttggtttaatggacctgttgtgtcctctgtgttgtacccaaaactcttctgcagcagtatggcttgaatccttatgaagtttgatatttgaacttaaaagtctgctcattatgtttttttctggttatatctcctaattaactgcctgggatcaaatttgattcgctggtgtttattggacccctcccaggttcttgctttctaccgtttcttgctgaatgttaacttgattctgtcaggctcagtttcccactatggcttacagcttaacgtgtttggtttgttgaatgttaacttggttttgtcaagctcagttttttactctggcttacagcataacatgtttgacttttggttttgctgctttgttattgggttctgggtagttcttgatgaatccaaaagatcatgtgcacagccatattatctatttaagcgatccaggttattactatgaaaggatgccttctagctaaggagtagttaggttttttcttcaaggttaaattttctcgatgctctagtgttcctgtgaccataatcataataattcctttgaaagctctatggtccctggaagcagggcatacaatgcaagacagcaacttgatcacatcaactgaagtatacagggttctcttaactcttggtgacttcggtttaatggaccggttgtactcgtgttctatccgtaaccgttgtgatgtcttgtgtgtttggttgcgggatagctgggaccacgacgtttccgtctaattctgatggatagctatagacggcactgagatggttatattataacctctgatcctgaactctacgagatcgtctcatccgtcattgccaccaaatacaccattaaatta

SEQ ID NO: 18 - DNA, 5527 bp, Artificial Sequence
  derived from Streptomyces viridochromogenes and Zea mays
ggaaaaccaaaacaacgaataagcaaactgcaggaaaagtatgcagtggaaaccaacccagattcggacgataggaaagtatcaagtgaatgatttgccaggaaaaggagaggggtaaaaaggggcgaagatttagaagatctaaagcacaagaaccagagattagattgaacaatagggaacttggagcatcctttttttcttcagggaaaaactgaaaatccaaaccatgttgagcaaaaccgagtgggattggaaaccaaaaaacccgagataaagaaactcgagaaaaagcatgaaatcgaaaccaacttcagtaaaacaaaaggaggacagaaaagaaagtcggaagctataaagaatacattaacattcagtgaaacagcatgctgtcttcttctttttttatgcacaacagagcatacatatataccttcccaggctgaggacttggcggaggagagccgcggataggttggcggtgcagacggtctggacgggcccgaagacggagacgaacagcgggcccttcctgcccaggcaccacgcttggaacgccaagcacgcgccaaccgcggccccgccgaggacgacgatccccgcgacaagcgtggcgtcgatcctgggcgaccccaagccgaggaacctcccttccaggacgagccgtaggacggcggtgagagaggcacccgtcgcggaggtggcgcagcacaaggtgagcagcgcggggaaggcggcgagcgtggcggcctgcaggacggtgacgagcgcgaagacggtgacgccggcgacgaggcagcagcagccgaggttccagtcgtaggaggaagccggaccaaaccgggcaatgcaacctgcagatgcactagacggaggtaacgaggaggaggagaaaacagagcaagagcaggcggagagaagatagagcaaaacacgagtgaggcacagcgtaagcactcggtagaagtctccagaggcgaggtgcgcacaggagaacagatgagtaaagtcagccaaggatgcacgatccaacggctacgaatttttggagtgacgtggataggctcaaaggcgccatttccatccggctttatagtattttaaaaaaattcattttcctccctctagtgtgtgcggaggcgtgagcccgtttaacggcgttgagaagtctaacggacaccaaccacaaccaggaaccagcgccggccgcgccgccgagtgaagcagactgcatacggcacggcgcggcatctctctggctgcctctcgagagttccgcccccaccttcccgcggtagcgtggtggtttcgctttccgctgtcggcatccggaagttgcgtggcagagtggacggagacgaggccgggtcctccagctcctctcaaacgtcacggcaccggcatccggcagccagcgcggtccttcccaaccactcgttcccaacccatcccccttcctcgcccgccgtcataaatagccagccccatccccagcttctttccccaacctcatcttctctccttttgctctgaacgcacacaccgcccggtctccgatctccgatccccgatcccctcgtcgatcctaggtacggcgaccatcctaccccccccccccccccctctctctctgccttctctagatcggcgatccgatccatgcttacttggttagggcctgctaactatgttcatgtttgcgttagatccgtgcatggacgcgatctgtacacaccagacgcgttctgattgctagctaactcgccagtacctgggaatcctgggatggctgtagccggccccgcacgcagacgggaccgatttcatgattctctatttttttctttgtttcgttgcctagggtttcgttcgatcgatccgcgttattctttatttccatatattctggtacgatgttgatacggttcgaccgtgctgcttacgttctgtgcgcttgtttgccgggtcatttttaccttgccttttttgtatggtttggttgtggcgatgtggtctggtcgggctgtcgttctagatcggagtagagtgctgtttcaaactgtctagcggatctattagatttggatctgcatgtgtgacatatatcttcgtagttaagatgatgcatctgtatgtgtgacatgcggatctattagatttggatctgtatgtgtgacatatatcttcgtagttgagatgatgcatctgtatgtgtgacatatatcttcgtagttaagattatgcatggaaatatcaatcctttagataaggacgggtatacttgttgctgtgggttttactggtacttcgatagatgcatatacatgatctaacatgcttagatacatgaagtaacatgctgctacggtttaataattcttgagttgatttttactggtacttagatagatgtatatacatgcttagatacatgaagtaacatgctcctacagttcctttaatcattattgagtacctatatattctaataaatcagtatgttttaaattattttgattttactggtacttagatagatgtatatatacatgctcaaacatgcttagatacatgaagtaacatgctgctacggtttagtcattattgagtgcctatatattctaataaatcagtatgttttaaattattttgattttactggtacttagatagatgtatatatacatgctcaaacatgcttagatacatgaagtaatatgctactacggtttaattgttcttgagtacctatatattctaataaatcagtatgttttaaattatttcgattttactggtacttagatagatgtatatatacatgcttagatacatgaagtaacatgctactacggtttaattgttcttgaatacctatatattctaataaatcagtatgttttaaattatttcgattttactggtacttagatagatgtatatatacatgctcgaacatgcttagatacatgaagtaacatgctacatatatattataataaatcagtatgtcttaaattattttgattttactggtacttagatagatgtatatacatgctcaaacatgcttagatacatgaagtaacatgctactacggtttaatcattattgagtacctatatattctaataaatcagtatgttttcaattgttttgattttactggtacttagatatatgtatatatacatgctcgaacatgcttagatacgtgaagtaacatgctactatggttaattgttcttgagtacctatatattctaataaatcagtatgttttaaattatttcgattttactggtacttagatagatgtatatatacatgctcgaacatgcttagatacatgaagtaacatgctactacggtttaatcgttcttgagtacctatatattctaataaatcagtatgtcttaaattatcttgattttactggtacttagatagatgtatatacatgcttagatacatgaagtaacatgctactatgatttaatcgttcttgagtacctatatattctaataaatcagtatgtttttaattattttgattttactggtacttagatagatgtatatatacatgctcgaacatgcttagatacatgaagtaacatgctactacggtttaatcattcttgagtacctatatattctaataaatcagtatgtttttaattattttgatattactggtacttaacatgtttagatacatcatatagcatgcacatgctgctactgtttaatcattcgtgaatacctatatattctaatatatcagtatgtcttctaattattatgattttgatgtacttgtatggtggcatatgctgcagctatgtgtagattttgaatacccagtgtgatgagcatgcatggcgccttcatagttcatatgctgtttatttcctttgagactgttcttttttgttgatagtcaccctgttgtttggtgattcttatccagatgtccccagagaggaggccagtggagatcaggccagccaccgccgccgacatggccgccgtgtgcgacatcgtgaaccactacatcgagacctccaccgtgaacttcaggaccgagccacagaccccacaggagtggatcgacgacctcgagaggctccaggacagatacccctggctcgtggccgaggtggagggcgtggtggccggcatcgcctacgccggcccctggaaagctaggaacgcctacgactggaccgtggagtccaccgtgtacgtgtcccacaggcaccagaggctcggcctcggctccaccctctacacccacctcctcaagtctatggaggcccagggcttcaagtccgtggtggccgtgatcggcctaccaaacgacccatccgtgaggctccacgaggccctcggctacaccgcgagaggcaccctcagggccgccggctacaagcacggcggctggcacgacgtgggcttctggcagagggacttcgagctgccagccccaccaaggccagtgaggccagtgacccagatttgagccaaggttcaattaagctgctgctgtacctgggtatctgcgtcgtctggtgccctctggtgtacctctatatggatctcgtcgtctaataaacatctgtggtttgtgtgtcatcaatcgtggttgtggcttcgttggtttaatggacctgttgtgtcctctgtgttgtacccaaaactcttctgcagcagtatggcttgaatccttatgaagtttgatatttgaacttaaaagtctgctcattatgtttttttctggttatatctcctaattaactgcctgggatcaaatttgattcgctggtgtttattggacccctcccaggttcttgctttctaccgtttcttgctgaatgttaacttgattctgtcaggctcagtttcccactatggcttacagcttaacgtgtttggtttgttgaatgttaacttggttttgtcaagctcagttttttactctggcttacagcataacatgtttgacttttggttttgctgctttgttattgggttctgggtagttcttgatgaatccaaaagatcatgtgcacagccatattatctatttaagcgatccaggttattactatgaaaggatgccttctagctaaggagtagttaggttttttcttcaaggttaaattttctcgatgctctagtgttcctgtgaccataatcataataattcctttgaaagctctatggtccctggaagcagggcatacaatgcaagacagcaacttgatcacatcaactgaagtatacagggttctcttaactcttggtgacttcggtttaatggaccggttgtactcgtgttctatccgtaaccgttgtgatgtcttgtgtgtttggttgcgggatagctgggaccacgacgtttccgtctaattctgatggatagctatagacggcactgagatggttatattataacctctgatcctgaactctacgagatcgtctcatccgtcattgccaccaaatacaccattaaatta

SEQ ID NO: 19 - DNA, 6067 bp, Artificial Sequence
  derived from Streptomyces viridochromogenes and Zea mays
agctgcttgtggggaccagacaaaaaaggaatggtgcagaattgttaggcgcacctaccaaaagcaactttgcctttattgcaaagataaagcagattcctctagtacaagtggggaacaaaataacgtggaaaagagctgtcctgacagcccactcactattgcgtttgacgaacgcagtgacgaccacaaaactcgagacttttcaacaaagggtattatccggaaacctcctcggattccattgcccagctatctgtcactttattgtgaagatagtggaaaaggaaggtggctcctacaaatgccatcattgcgataaaggaaaggctatcgttgaagatgcctctgccgacagtggtcccaaagatggacccccacccacgaggagcatcgtggaaaaagaagacgttccaaccacgtcttcaaagcaagtggattgatgtgatatctccactgacgtaagggttgacgaacaatcccactatccttctgcctaattagctaacggacccggaaaaccaaaacaacgaataagcaaactgcaggaaaagtatgcagtggaaaccaacccagattcggacgataggaaagtatcaagtgaatgatttgccaggaaaaggagaggggtaaaaaggggcgaagatttagaagatctaaagcacaagaaccagagattagattgaacaatagggaacttggagcatcctttttttcttcagggaaaaactgaaaatccaaaccatgttgagcaaaaccgagtgggattggaaaccaaaaaacccgagataaagaaactcgagaaaaagcatgaaatcgaaaccaacttcagtaaaacaaaaggaggacagaaaagaaagtcggaagctataaagaatacattaacattcagtgaaacagcatgctgtcttcttctttttttatgcacaacagagcatacatatataccttcccaggctgaggacttggcggaggagagccgcggataggttggcggtgcagacggtctggacgggcccgaagacggagacgaacagcgggcccttcctgcccaggcaccacgcttggaacgccaagcacgcgccaaccgcggccccgccgaggacgacgatccccgcgacaagcgtggcgtcgatcctgggcgaccccaagccgaggaacctcccttccaggacgagccgtaggacggcggtgagagaggcacccgtcgcggaggtggcgcagcacaaggtgagcagcgcggggaaggcggcgagcgtggcggcctgcaggacggtgacgagcgcgaagacggtgacgccggcgacgaggcagcagcagccgaggttccagtcgtaggaggaagccggaccaaaccgggcaatgcaacctgcagatgcactagacggaggtaacgaggaggaggagaaaacagagcaagagcaggcggagagaagatagagcaaaacacgagtgaggcacagcgtaagcactcggtagaagtctccagaggcgaggtgcgcacaggagaacagatgagtaaagtcagccaaggatgcacgatccaacggctacgaatttttggagtgacgtggataggctcaaaggcgccatttccatccggctttatagtattttaaaaaaattcattttcctccctctagtgtgtgcggaggcgtgagcccgtttaacggcgttgagaagtctaacggacaccaaccacaaccaggaaccagcgccggccgcgccgccgagtgaagcagactgcatacggcacggcgcggcatctctctggctgcctctcgagagttccgcccccaccttcccgcggtagcgtggtggtttcgctttccgctgtcggcatccggaagttgcgtggcagagtggacggagacgaggccgggtcctccagctcctctcaaacgtcacggcaccggcatccggcagccagcgcggtccttcccaaccactcgttcccaacccatcccccttcctcgcccgccgtcataaatagccagccccatccccagcttctttccccaacctcatcttctctccttttgctctgaacgcacacaccgcccggtctccgatctccgatccccgatcccctcgtcgatcctaggtacggcgaccatcctaccccccccccccccccctctctctctgccttctctagatcggcgatccgatccatgcttacttggttagggcctgctaactatgttcatgtttgcgttagatccgtgcatggacgcgatctgtacacaccagacgcgttctgattgctagctaactcgccagtacctgggaatcctgggatggctgtagccggccccgcacgcagacgggaccgatttcatgattctctatttttttctttgtttcgttgcctagggtttcgttcgatcgatccgcgttattctttatttccatatattctggtacgatgttgatacggttcgaccgtgctgcttacgttctgtgcgcttgtttgccgggtcatttttaccttgccttttttgtatggtttggttgtggcgatgtggtctggtcgggctgtcgttctagatcggagtagagtgctgtttcaaactgtctagcggatctattagatttggatctgcatgtgtgacatatatcttcgtagttaagatgatgcatctgtatgtgtgacatgcggatctattagatttggatctgtatgtgtgacatatatcttcgtagttgagatgatgcatctgtatgtgtgacatatatcttcgtagttaagattatgcatggaaatatcaatcctttagataaggacgggtatacttgttgctgtgggttttactggtacttcgatagatgcatatacatgatctaacatgcttagatacatgaagtaacatgctgctacggtttaataattcttgagttgatttttactggtacttagatagatgtatatacatgcttagatacatgaagtaacatgctcctacagttcctttaatcattattgagtacctatatattctaataaatcagtatgttttaaattattttgattttactggtacttagatagatgtatatatacatgctcaaacatgcttagatacatgaagtaacatgctgctacggtttagtcattattgagtgcctatatattctaataaatcagtatgttttaaattattttgattttactggtacttagatagatgtatatatacatgctcaaacatgcttagatacatgaagtaatatgctactacggtttaattgttcttgagtacctatatattctaataaatcagtatgttttaaattatttcgattttactggtacttagatagatgtatatatacatgcttagatacatgaagtaacatgctactacggtttaattgttcttgaatacctatatattctaataaatcagtatgttttaaattatttcgattttactggtacttagatagatgtatatatacatgctcgaacatgcttagatacatgaagtaacatgctacatatatattataataaatcagtatgtcttaaattattttgattttactggtacttagatagatgtatatacatgctcaaacatgcttagatacatgaagtaacatgctactacggtttaatcattattgagtacctatatattctaataaatcagtatgttttcaattgttttgattttactggtacttagatatatgtatatatacatgctcgaacatgcttagatacgtgaagtaacatgctactatggttaattgttcttgagtacctatatattctaataaatcagtatgttttaaattatttcgattttactggtacttagatagatgtatatatacatgctcgaacatgcttagatacatgaagtaacatgctactacggtttaatcgttcttgagtacctatatattctaataaatcagtatgtcttaaattatcttgattttactggtacttagatagatgtatatacatgcttagatacatgaagtaacatgctactatgatttaatcgttcttgagtacctatatattctaataaatcagtatgtttttaattattttgattttactggtacttagatagatgtatatatacatgctcgaacatgcttagatacatgaagtaacatgctactacggtttaatcattcttgagtacctatatattctaataaatcagtatgtttttaattattttgatattactggtacttaacatgtttagatacatcatatagcatgcacatgctgctactgtttaatcattcgtgaatacctatatattctaatatatcagtatgtcttctaattattatgattttgatgtacttgtatggtggcatatgctgcagctatgtgtagattttgaatacccagtgtgatgagcatgcatggcgccttcatagttcatatgctgtttatttcctttgagactgttcttttttgttgatagtcaccctgttgtttggtgattcttatccagatccagatcttcgagatcctaaaccatgtccccagagaggaggccagtggagatcaggccagccaccgccgccgacatggccgccgtgtgcgacatcgtgaaccactacatcgagacctccaccgtgaacttcaggaccgagccacagaccccacaggagtggatcgacgacctcgagaggctccaggacagatacccctggctcgtggccgaggtggagggcgtggtggccggcatcgcctacgccggcccctggaaagctaggaacgcctacgactggaccgtggagtccaccgtgtacgtgtcccacaggcaccagaggctcggcctcggctccaccctctacacccacctcctcaagtctatggaggcccagggcttcaagtccgtggtggccgtgatcggcctaccaaacgacccatccgtgaggctccacgaggccctcggctacaccgcgagaggcaccctcagggccgccggctacaagcacggcggctggcacgacgtgggcttctggcagagggacttcgagctgccagccccaccaaggccagtgaggccagtgacccagatttgagccaaggttcaattaagctgctgctgtacctgggtatctgcgtcgtctggtgccctctggtgtacctctatatggatctcgtcgtctaataaacatctgtggtttgtgtgtcatcaatcgtggttgtggcttcgttggtttaatggacctgttgtgtcctctgtgttgtacccaaaactcttctgcagcagtatggcttgaatccttatgaagtttgatatttgaacttaaaagtctgctcattatgtttttttctggttatatctcctaattaactgcctgggatcaaatttgattcgctggtgtttattggacccctcccaggttcttgctttctaccgtttcttgctgaatgttaacttgattctgtcaggctcagtttcccactatggcttacagcttaacgtgtttggtttgttgaatgttaacttggttttgtcaagctcagttttttactctggcttacagcataacatgtttgacttttggttttgctgctttgttattgggttctgggtagttcttgatgaatccaaaagatcatgtgcacagccatattatctatttaagcgatccaggttattactatgaaaggatgccttctagctaaggagtagttaggttttttcttcaaggttaaattttctcgatgctctagtgttcctgtgaccataatcataataattcctttgaaagctctatggtccctggaagcagggcatacaatgcaagacagcaacttgatcacatcaactgaagtatacagggttctcttaactcttggtgacttcggtttaatggaccggttgtactcgtgttctatccgtaaccgttgtgatgtcttgtgtgtttggttgcgggatagctgggaccacgacgtttccgtctaattctgatggatagctatagacggcactgagatggttatattataacctctgatcctgaactctacgagatcgtctcatccgtcattgccaccaaatacaccattaaatta

SEQ ID NO: 20 - DNA, 6042 bp, Artificial Sequence
  derived from Streptomyces viridochromogenes and Zea mays
agctgcttgtggggaccagacaaaaaaggaatggtgcagaattgttaggcgcacctaccaaaagcaactttgcctttattgcaaagataaagcagattcctctagtacaagtggggaacaaaataacgtggaaaagagctgtcctgacagcccactcactattgcgtttgacgaacgcagtgacgaccacaaaactcgagacttttcaacaaagggtattatccggaaacctcctcggattccattgcccagctatctgtcactttattgtgaagatagtggaaaaggaaggtggctcctacaaatgccatcattgcgataaaggaaaggctatcgttgaagatgcctctgccgacagtggtcccaaagatggacccccacccacgaggagcatcgtggaaaaagaagacgttccaaccacgtcttcaaagcaagtggattgatgtgatatctccactgacgtaagggttgacgaacaatcccactatccttctgcctaattagctaacggacccggaaaaccaaaacaacgaataagcaaactgcaggaaaagtatgcagtggaaaccaacccagattcggacgataggaaagtatcaagtgaatgatttgccaggaaaaggagaggggtaaaaaggggcgaagatttagaagatctaaagcacaagaaccagagattagattgaacaatagggaacttggagcatcctttttttcttcagggaaaaactgaaaatccaaaccatgttgagcaaaaccgagtgggattggaaaccaaaaaacccgagataaagaaactcgagaaaaagcatgaaatcgaaaccaacttcagtaaaacaaaaggaggacagaaaagaaagtcggaagctataaagaatacattaacattcagtgaaacagcatgctgtcttcttctttttttatgcacaacagagcatacatatataccttcccaggctgaggacttggcggaggagagccgcggataggttggcggtgcagacggtctggacgggcccgaagacggagacgaacagcgggcccttcctgcccaggcaccacgcttggaacgccaagcacgcgccaaccgcggccccgccgaggacgacgatccccgcgacaagcgtggcgtcgatcctgggcgaccccaagccgaggaacctcccttccaggacgagccgtaggacggcggtgagagaggcacccgtcgcggaggtggcgcagcacaaggtgagcagcgcggggaaggcggcgagcgtggcggcctgcaggacggtgacgagcgcgaagacggtgacgccggcgacgaggcagcagcagccgaggttccagtcgtaggaggaagccggaccaaaccgggcaatgcaacctgcagatgcactagacggaggtaacgaggaggaggagaaaacagagcaagagcaggcggagagaagatagagcaaaacacgagtgaggcacagcgtaagcactcggtagaagtctccagaggcgaggtgcgcacaggagaacagatgagtaaagtcagccaaggatgcacgatccaacggctacgaatttttggagtgacgtggataggctcaaaggcgccatttccatccggctttatagtattttaaaaaaattcattttcctccctctagtgtgtgcggaggcgtgagcccgtttaacggcgttgagaagtctaacggacaccaaccacaaccaggaaccagcgccggccgcgccgccgagtgaagcagactgcatacggcacggcgcggcatctctctggctgcctctcgagagttccgcccccaccttcccgcggtagcgtggtggtttcgctttccgctgtcggcatccggaagttgcgtggcagagtggacggagacgaggccgggtcctccagctcctctcaaacgtcacggcaccggcatccggcagccagcgcggtccttcccaaccactcgttcccaacccatcccccttcctcgcccgccgtcataaatagccagccccatccccagcttctttccccaacctcatcttctctccttttgctctgaacgcacacaccgcccggtctccgatctccgatccccgatcccctcgtcgatcctaggtacggcgaccatcctaccccccccccccccccctctctctctgccttctctagatcggcgatccgatccatgcttacttggttagggcctgctaactatgttcatgtttgcgttagatccgtgcatggacgcgatctgtacacaccagacgcgttctgattgctagctaactcgccagtacctgggaatcctgggatggctgtagccggccccgcacgcagacgggaccgatttcatgattctctatttttttctttgtttcgttgcctagggtttcgttcgatcgatccgcgttattctttatttccatatattctggtacgatgttgatacggttcgaccgtgctgcttacgttctgtgcgcttgtttgccgggtcatttttaccttgccttttttgtatggtttggttgtggcgatgtggtctggtcgggctgtcgttctagatcggagtagagtgctgtttcaaactgtctagcggatctattagatttggatctgcatgtgtgacatatatcttcgtagttaagatgatgcatctgtatgtgtgacatgcggatctattagatttggatctgtatgtgtgacatatatcttcgtagttgagatgatgcatctgtatgtgtgacatatatcttcgtagttaagattatgcatggaaatatcaatcctttagataaggacgggtatacttgttgctgtgggttttactggtacttcgatagatgcatatacatgatctaacatgcttagatacatgaagtaacatgctgctacggtttaataattcttgagttgatttttactggtacttagatagatgtatatacatgcttagatacatgaagtaacatgctcctacagttcctttaatcattattgagtacctatatattctaataaatcagtatgttttaaattattttgattttactggtacttagatagatgtatatatacatgctcaaacatgcttagatacatgaagtaacatgctgctacggtttagtcattattgagtgcctatatattctaataaatcagtatgttttaaattattttgattttactggtacttagatagatgtatatatacatgctcaaacatgcttagatacatgaagtaatatgctactacggtttaattgttcttgagtacctatatattctaataaatcagtatgttttaaattatttcgattttactggtacttagatagatgtatatatacatgcttagatacatgaagtaacatgctactacggtttaattgttcttgaatacctatatattctaataaatcagtatgttttaaattatttcgattttactggtacttagatagatgtatatatacatgctcgaacatgcttagatacatgaagtaacatgctacatatatattataataaatcagtatgtcttaaattattttgattttactggtacttagatagatgtatatacatgctcaaacatgcttagatacatgaagtaacatgctactacggtttaatcattattgagtacctatatattctaataaatcagtatgttttcaattgttttgattttactggtacttagatatatgtatatatacatgctcgaacatgcttagatacgtgaagtaacatgctactatggttaattgttcttgagtacctatatattctaataaatcagtatgttttaaattatttcgattttactggtacttagatagatgtatatatacatgctcgaacatgcttagatacatgaagtaacatgctactacggtttaatcgttcttgagtacctatatattctaataaatcagtatgtcttaaattatcttgattttactggtacttagatagatgtatatacatgcttagatacatgaagtaacatgctactatgatttaatcgttcttgagtacctatatattctaataaatcagtatgtttttaattattttgattttactggtacttagatagatgtatatatacatgctcgaacatgcttagatacatgaagtaacatgctactacggtttaatcattcttgagtacctatatattctaataaatcagtatgtttttaattattttgatattactggtacttaacatgtttagatacatcatatagcatgcacatgctgctactgtttaatcattcgtgaatacctatatattctaatatatcagtatgtcttctaattattatgattttgatgtacttgtatggtggcatatgctgcagctatgtgtagattttgaatacccagtgtgatgagcatgcatggcgccttcatagttcatatgctgtttatttcctttgagactgttcttttttgttgatagtcaccctgttgtttggtgattcttatccagatgtccccagagaggaggccagtggagatcaggccagccaccgccgccgacatggccgccgtgtgcgacatcgtgaaccactacatcgagacctccaccgtgaacttcaggaccgagccacagaccccacaggagtggatcgacgacctcgagaggctccaggacagatacccctggctcgtggccgaggtggagggcgtggtggccggcatcgcctacgccggcccctggaaagctaggaacgcctacgactggaccgtggagtccaccgtgtacgtgtcccacaggcaccagaggctcggcctcggctccaccctctacacccacctcctcaagtctatggaggcccagggcttcaagtccgtggtggccgtgatcggcctaccaaacgacccatccgtgaggctccacgaggccctcggctacaccgcgagaggcaccctcagggccgccggctacaagcacggcggctggcacgacgtgggcttctggcagagggacttcgagctgccagccccaccaaggccagtgaggccagtgacccagatttgagccaaggttcaattaagctgctgctgtacctgggtatctgcgtcgtctggtgccctctggtgtacctctatatggatctcgtcgtctaataaacatctgtggtttgtgtgtcatcaatcgtggttgtggcttcgttggtttaatggacctgttgtgtcctctgtgttgtacccaaaactcttctgcagcagtatggcttgaatccttatgaagtttgatatttgaacttaaaagtctgctcattatgtttttttctggttatatctcctaattaactgcctgggatcaaatttgattcgctggtgtttattggacccctcccaggttcttgctttctaccgtttcttgctgaatgttaacttgattctgtcaggctcagtttcccactatggcttacagcttaacgtgtttggtttgttgaatgttaacttggttttgtcaagctcagttttttactctggcttacagcataacatgtttgacttttggttttgctgctttgttattgggttctgggtagttcttgatgaatccaaaagatcatgtgcacagccatattatctatttaagcgatccaggttattactatgaaaggatgccttctagctaaggagtagttaggttttttcttcaaggttaaattttctcgatgctctagtgttcctgtgaccataatcataataattcctttgaaagctctatggtccctggaagcagggcatacaatgcaagacagcaacttgatcacatcaactgaagtatacagggttctcttaactcttggtgacttcggtttaatggaccggttgtactcgtgttctatccgtaaccgttgtgatgtcttgtgtgtttggttgcgggatagctgggaccacgacgtttccgtctaattctgatggatagctatagacggcactgagatggttatattataacctctgatcctgaactctacgagatcgtctcatccgtcattgccaccaaatacaccattaaatta

SEQ ID NO: 21 - DNA, 552 bp, Artificial Sequence
  derived from Streptomyces viridochromogenes
atgtctccggagaggagaccagttgagattaggccagctacagcagctgatatggccgcggtttgtgatatcgttaaccattacattgagacgtctacagtgaactttaggacagagccacaaacaccacaagagtggattgatgatctagagaggttgcaagatagatacccttggttggttgctgaggttgagggtgttgtggctggtattgcttacgctgggccctggaaggctaggaacgcttacgattggacagttgagagtactgtttacgtgtcacataggcatcaaaggttgggcctaggctccacattgtacacacatttgcttaagtctatggaggcgcaaggttttaagtcagtggttgctgttataggccttccaaacgatccatctgttaggttgcatgaggctctaggatacacagcgcggggtacactgcgcgcagctggatacaagcatggtggatggcatgatgttggtttttggcaaagggattttgagttgccagctcctccaaggccagtgaggccagttacccagatctga

SEQ ID NO: 22 - DNA, 1343 bp, Artificial Sequence
  derived from Streptomyces viridochromogenes and Zea mays
agtcaaagattcaaatagaggacctaacagaactcgccgtaaagactggcgaacagttcatacagagtctcttacgactcaatgacaagaagaaaatcttcgtcaacttggtggagcacgacacgctagtctactccaaaaatatcaaagatacagtctcagaagaccaaagggcaattgagacttttcaacaaagggtaatatccggaaacctcctcggattccattgcccagctatctgtcacttaattgtgaagatagtggaaaaggaaggtggctcctacaaatgccatcattgcgataaaggaaaggccatcgttgaagatgcctctgccgacagtggtcccaaagatggacccccacccacgaggagcatcgtggtaaaagaagacgttccaaccacgtcttcaaagcaagtggattgatgtgatatctccactgacgtaagggatgacgcacaatcccactatccttcgcaagacccttcctctatataaggaagttcatttcatttggagaggataattatccaccatgtctccggagaggagaccagttgagattaggccagctacagcagctgatatggccgcggtttgtgatatcgttaaccattacattgagacgtctacagtgaactttaggacagagccacaaacaccacaagagtggattgatgatctagagaggttgcaagatagatacccttggttggttgctgaggttgagggtgttgtggctggtattgcttacgctgggccctggaaggctaggaacgcttacgattggacagttgagagtactgtttacgtgtcacataggcatcaaaggttgggcctaggctccacattgtacacacatttgcttaagtctatggaggcgcaaggttttaagtcagtggttgctgttataggccttccaaacgatccatctgttaggttgcatgaggctctaggatacacagcgcggggtacactgcgcgcagctggatacaagcatggtggatggcatgatgttggtttttggcaaagggattttgagttgccagctcctccaaggccagtgaggccagttacccagatctgactaagatcgttcaaacatttggcaataaagtttcttaagattgaatcctgttgccggtcttgcgatgattatcatataatttctgttgaattacgttaagcatgtaataattaacatgtaatgcatgacgttatttatgagatgggtttttatgattagagtcccgcaattatacatttaatacgcgatagaaaacaaaatatagcgcgcaaactaggataaattatcgcgcgcggtgtcatctatgttactagatc

SEQ ID NO: 23 - DNA, 6135 bp, Artificial Sequence
  derived from Streptomyces viridochromogenes and Zea mays
agctgcttgtggggaccagacaaaaaaggaatggtgcagaattgttaggcgcacctaccaaaagcatctttgcctttattgcaaagataaagcagattcctctagtacaagtggggaacaaaataacgtggaaaagagctgtcctgacagcccactcactattgcgtttgacgaacgcagtgacgaccacaaaactcgagacttttcaacaaagggtaatatccggaaacctcctcggattccattgcccagctatctgtcactttattgtgaagatagtggaaaaggaaggtggctcctacaaatgccatcattgcgataaaggaaaggctatcgttgaagatgcctctgccgacagtggtcccaaagatggacccccacccacgaggagcatcgtggaaaaagaagacgttccaaccacgtcttcaaagcaagtggattgatgtgatatctccactgacgtaagggatgacgaacaatcccactatccttctgccggaccctggaaaaccaaaacaacgaataagcaaactgcaggaaaagtatgcagtggaaaccaacccagattcggacgataggaaagtatcaagtgaatgatttgccaggaaaaggagaggggtaaaaaggggcgaagatttagaagatctaaagcacaagaaccagagattagattgaacaatagggaacttggagcatcctttttttcttcagggaaaaactgaaaatccaaaccatgttgagcaaaaccgagtgggattggaaaccaaaaaacccgagataaagaaactcgagaaaaagcatgaaatcgaaaccaacttcagtaaaacaaaaggaggacagaaaagaaagtcggaaggtataaagaatacattaacattcagtgaaacagcatgctgtcttcttctttttttatgcacaacagagcatacatatataccttcccaggctgaggacttggcggaggagagccgcggagaggttggcggtgcagacggtctggacgggcccgaagacggagacgaacagcgggcccttcctgcccaggcaccacgcttggaacgccaagcacgcgccaaccgcggccccgccgaggacgacgatccccgcgacaagcgtggcgtcgatcctgggcgaccccaagccgaggaacctcccttccaggacgagccgcaggacggcggtgagagaggcacccgtcgcggaggtggcgcagcacaaggtgagcagcgcggggaaggcggcgagcgtggcggcctgcaggacggtgacgagcgcgaagacggtgacgccggcgacgaggcagcagcagccgaggatccagtcgtaggaggaagccggaccaaaccgggcaatgcaacctgcagatgcactagacggaggaaacgaggaggaggagaaaacagagcaagagcaggcggagagaagatagagcaaaacacgagtgaggcacagcgtaagcactcggtagaagtctccagaggcgaggtgcgcacaggagaacagatgagtaaagtcagccaaggatccacgatccaacggctacgaatttttggagtgacgtggataggctcaaaggcgccatttccatccggctttatagtattttaaaaaaattcattttcctccctctagtgtgtgcggaggcgtgagcccgtttaacggcgttgagaagtctaacggacaccaaccacaaccaggaaccagcgccggccgcgccgccgagtgaagcagactgcatacggcacggcgcggcatctctctggctgcctctcgagagttccgcccccaccttcccgcggtagcgtggtggtttcgctttccgctgtcggcatccggaagttgcgtggcagagtggacggagacgaggccgggtcctccagctcctctcaaacgtcacggcaccggcatccggcagccagcgcggtccttcccaaccactcgttcccaacccatcccccttcctcgcccgccgtcataaatagccagccccatccccagcttctttccccaacctcatcttctctccttttgctctgaacgcacacaccgcccggtctccgatctccgatccccgatcccctcgtcgatcctaggtacggcgaccatcctcccccccccccccccccctctctctctgccttctctagatcggcgatccgatccatgcttacttggttagggcctgctaactatgttcatgtttgcgttagatccgtgcatggacgcgatctgtacacaccagacgcgttctgattgctagctaactcgccagtacctgggaatcctgggatggctgtagccggccccgcacgcagacgggaccgatttcatgattctctatttttttctttgtttcgttgcctagggtttcgttcgatcgatccgcgttattctttatttccatatattctggtacgatgttgatacggttcgaccgtgctgcttacgttctgtgcgcttgtttgccgggtcatttttaccttgccttttttgtatggtttggttgtggcgatgtggtctggtcgggctgtcgttctagatcggagtagagtgctgtttcaaactgtctagcggatctattagatttggatctgcatgtgtgacatatatcttcgtagttaagatgatgcatctgtatgtgtgacatgcggatctattagatttggatctgtatgtgtgacatatatcttcgtagttgagatgatgcatctgtatgtgtgacatatatcttcgtagttaagattatgcatggaaatatcaatcctttagataaggacgggtatacttgttgctgtgggttttactggtacttcgatagatgcatatacatgatctaacatgcttagatacatgaagtaacatgctgctacggtttaataattcttgagttgatttttactggtacttagatagatgtatatacatgcttagatacatgaagtaacatgctcctacagttcctttaatcattattgagtacctatatattctaataaatcagtatgttttaaattattttgattttactggtacttagatagatgtatatatacatgctcaaacatgcttagatacatgaagtaacatgctgctacggtttagtcattattgagtgcctatatattctaataaatcagtatgttttaaattattttgattttactggtacttagatagatgtatatatacatgctcaaacatgcttagatacatgaagtaatatgctactacggtttaattgttcttgagtacctatatattctaataaatcagtatgttttaaattatttcgattttactggtacttagatagatgtatatatacatgcttagatacatgaagtaacatgctactacggtttaattgttcttgaatacctatatattctaataaatcagtatgttttaaattatttcgattttactggtacttagatagatgtatatatacatgctcgaacatgcttagatacatgaagtaacatgctacatatatattataataaatcagtatgtcttaaattattttgattttactggtacttagatagatgtatatacatgctcaaacatgcttagatacatgaagtaacatgctactacggtttaatcattattgagtacctatatattctaataaatcagtatgttttcaattgttttgattttactggtacttagatatatgtatatatacatgctcgaacatgcttagatacgtgaagtaacatgctactatggttaattgttcttgagtacctatatattctaataaatcagtatgttttaaattatttcgattttactggtacttagatagatgtatatatacatgctcgaacatgcttagatacatgaagtaacatgctactacggtttaatcgttcttgagtacctatatattctaataaatcagtatgtcttaaattatcttgattttactggtacttagatagatgtatatacatgcttagatacatgaagtaacatgctactatgatttaatcgttcttgagtacctatatattctaataaatcagtatgtttttaattattttgattttactggtacttagatagatgtatatatacatgctcgaacatgcttagatacatgaagtaacatgctactacggtttaatcattcttgagtacctatatattctaataaatcagtatgtttttaattattttgatattactggtacttaacatgtttagatacatcatatagcatgcacatgctgctactgtttaatcattcgtgaatacctatatattctaatatatcagtatgtcttctaattattatgattttgatgtacttgtatggtggcatatgctgcagctatgtgtagattttgaatacccagtgtgatgagcatgcatggcgccttcatagttcatatgctgtttatttcctttgagactgttcttttttgttgatagtcaccctgttgtttggtgattcttatgcagatccagatcttcgtatttttacaacaattaccaacaacaacaaacaacaaacaacattacaattactatttacataaaccatggtctaattatccaccatgtctccggagaggagaccagttgagattaggccagctacagcagctgatatggccgcggtttgtgatatcgttaaccattacattgagacgtctacagtgaactttaggacagagccacaaacaccacaagagtggattgatgatctagagaggttgcaagatagatacccttggttggttgctgaggttgagggtgttgtggctggtattgcttacgctgggccctggaaggctaggaacgcttacgattggacagttgagagtactgtttacgtgtcacataggcatcaaaggttgggcctaggctccacattgtacacacatttgcttaagtctatggaggcgcaaggttttaagtcagtggttgctgttataggccttccaaacgatccatctgttaggttgcatgaggctctaggatacacagcgcggggtacactgcgcgcagctggatacaagcatggtggatggcatgatgttggtttttggcaaagggattttgagttgccagctcctccaaggccagtgaggccagttacccagatctgagagctcgccaaggttcaattaagctgctgctgtacctgggtatctgcgtcgtctggtgccctctggtgtacctctatatggatgtcgtcgtctaataaacatctgtggtttgtgtgtcatgaatcgtggttgtggcttcgttggtttaatggacctgttgtgtcctctgtgttgtacccaaaactcttctgcagcagtatggcttgaatccttatgaagtttgatatttgaacttaaaagtctgctcattatgtttttttctggttatatctcctaattaactgcctgggatcaaatttgattcgctggtgtttattggacccctcccaggttcttgctttctaccgtttcttgctgaatgttaacttgattctgtcaggctcagtttcccactatggcttacagcttaacgtgtttggtttgttgaatgttaacttggttttgtcaagctcagttttttactctggcttacagcataacatgtttgacttttggttttgctgctttgttattgggttctgggtagttcttgatgaatccaaaagatcatgtgcacagccatattatctatttaagcgatccaggttattactatgaaaggatgccttctagctaaggagtagttaggttttttcttcaaggttaaattttctcgatgctctagtgttcctgtgaccataatcataataattcctttgaaagctctatggtccctggaagcagggcatacaatgcaagacagcaacttgatcacatcaactgaagtatacagggttctcttaactcttggtgacttcggtttaatggaccggttgtactcgtgttctatccgtaaccgttgtgatgtcttgtgtgtttggttgcgggatagctgggaccacgacgtttccgtctaattctgatggatagctatagacggcactgagatggttatattataacctctgatcctgaactctacgagatcgtctcatccgtcattgccaccaaatacaccattaaatta

SEQ ID NO: 24 - DNA, 22 bp, Artificial Sequence
  derived from Streptomyces viridochromogenes
gcgacatcgtgaaccactacat

SEQ ID NO: 25 - DNA, 19 bp, Artificial Sequence
  derived from Streptomyces viridochromogenes
gctcgaggtcgtcgatcca

SEQ ID NO: 26 - DNA, 21 bp, Artificial Sequence
  derived from Streptomyces viridochromogenes
ccaccgtgaacttccgcaccg

SEQ ID NO: 27 - DNA, 17 bp, Artificial Sequence
  derived from Streptomyces viridochromogenes
gcgtcaggctgcacgaa

SEQ ID NO: 28 - DNA, 20 bp, Artificial Sequence
  derived from Streptomyces viridochromogenes
cgaagtccctctgccagaag

SEQ ID NO: 29 - DNA, 22 bp, Artificial Sequence
  derived from Streptomyces viridochromogenes
ctacaagcacggcggctggcac

SEQ ID NO: 30 - DNA, 17 bp, Artificial Sequence
  derived from Streptomyces viridochromogenes
cgaggccctcggctaca

SEQ ID NO: 31 - DNA, 20 bp, Artificial Sequence
  derived from Streptomyces viridochromogenes
cgaagtccctctgccagaag

SEQ ID NO: 32 - DNA, 22 bp, Artificial Sequence
  derived from Streptomyces viridochromogenes
ctacaagcacggcggctggcac

SEQ ID NO: 33 - DNA, 20 bp, Artificial Sequence
  derived from Streptomyces viridochromogenes
tgagggtgttgtggctggta

SEQ ID NO: 34 - DNA, 21 bp, Artificial Sequence
  derived from Streptomyces viridochromogenes
tgtccaatcgtaagcgttcct

SEQ ID NO: 35 - DNA, 22 bp, Artificial Sequence
  derived from Streptomyces viridochromogenes
cttccagggcccagcgtaagca